European Patent Application EP 4 186 920 A1, published May 31, 2023. Title: ULTRA-LONG ACTING INSULIN-FC FUSION PROTEINS AND METHODS OF USE. Applicant: AKSTON BIOSCIENCES CORPORATION. Application EP PCT/US2019/040010, filed June 28, 2019. The sequence listing filed with the application follows.

SEQUENCE LISTING (133 sequences)

SEQ ID NO: 1 - protein, 30 aa, synthetic construct
  REGION 1..30: note = hIns-B-chain
FVNQHLCGSHLVEALYLVCGERGFFYTPKT

SEQ ID NO: 2 - protein, 21 aa, synthetic construct
  REGION 1..21: note = hIns-A-chain
GIVEQCCTSICSLYQLENYCN

SEQ ID NO: 3 - protein, 86 aa, synthetic construct
  REGION 1..86: note = Human Proinsulin
FVNQHLCGSHLVEALYLVCGERGFFYTPKTRREAEDLQVGQVELGGGPGAGSLQPLALEGSLQKRGIVEQCCTSICSLYQLENYCN

SEQ ID NO: 4 - protein, 57 aa, synthetic construct
  REGION 1..57: note = Ins Polypeptide
FVNQHLCGSDLVEALYLVCGERGFFYTDPTGGGPRRGIVEQCCHSICSLYQLENYCN

SEQ ID NO: 5 - protein, 57 aa, synthetic construct
  REGION 1..57: note = Ins Polypeptide
FVNQHLCGSDLVEALALVCGERGFFYTDPTGGGPRRGIVEQCCHSICSLYQLENYCN

SEQ ID NO: 6 - protein, 58 aa, synthetic construct
  REGION 1..58: note = Ins Polypeptide
  SITE 10: note = X is not D
  SITE 45: note = X is not H
  SITE 58: note = X is absent or N
FVNQHLCGSXLVEALELVCGERGFHYGGGGGGSGGGGGIVEQCCXSTCSLDQLENYCX

SEQ ID NO: 7 - protein, 58 aa, synthetic construct
  REGION 1..58: note = Ins Polypeptide
  SITE 58: note = X is absent or N
FVNQHLCGSHLVEALELVCGERGFHYGGGGGGSGGGGGIVEQCCTSTCSLDQLENYCX

SEQ ID NO: 8 - protein, 57 aa, synthetic construct
  REGION 1..57: note = Ins Polypeptide
FVNQHLCGSHLVEALELVCGERGFHYGGGGGGSGGGGGIVEQCCTSTCSLDQLENYC

SEQ ID NO: 9 - protein, 58 aa, synthetic construct
  REGION 1..58: note = Ins Polypeptide
FVNQHLCGSHLVEALELVCGERGFHYGGGGGGSGGGGGIVEQCCTSTCSLDQLENYCN

SEQ ID NO: 10 - protein, 57 aa, synthetic construct
  REGION 1..57: note = Ins Polypeptide
  SITE 10: note = X is not D
  SITE 45: note = X is not H
FVNQHLCGSXLVEALALVCGERGFHYGGGGGGSGGGGGIVEQCCXSTCSLDQLENYC

SEQ ID NO: 11 - protein, 57 aa, synthetic construct
  REGION 1..57: note = Ins Polypeptide
FVNQHLCGSHLVEALALVCGERGFHYGGGGGGSGGGGGIVEQCCTSTCSLDQLENYC

SEQ ID NO: 12 - protein, 9 aa, synthetic construct
  REGION 1..9: note = Linker
GGGGAGGGG

SEQ ID NO: 13 - protein, 9 aa, synthetic construct
  REGION 1..9: note = Linker
GGGGSGGGG

SEQ ID NO: 14 - protein, 21 aa, synthetic construct
  REGION 1..21: note = Linker
GGGGGQGGGGQGGGGQGGGGG

SEQ ID NO: 15 - protein, 228 aa, synthetic construct
  REGION 1..228: note = Canine IgGA Fc Fragment
RCTDTPPCPVPEPLGGPSVLIFPPKPKDILRITRTPEVTCVVLDLGREDPEVQISWFVDGKEVHTAKTQSREQQFNGTYRVVSVLPIEHQDWLTGKEFKCRVNHIDLPSPIERTISKARGRAHKPSVYVLPPSPKELSSSDTVSITCLIKDFYPPDIDVEWQSNGQQEPERKHRMTPPQLDEDGSYFLYSKLSVDKSRWQQGDPFTCAVMHETLQNHYTDLSLSHSPG

SEQ ID NO: 16 - protein, 224 aa, synthetic construct
  REGION 1..224: note = Canine IgGB Fc Fragment
DCPKCPAPEMLGGPSVFIFPPKPKDTLLIARTPEVTCVVVDLDPEDPEVQISWFVDGKQMQTAKTQPREEQFNGTYRVVSVLPIGHQDWLKGKQFTCKVNNKALPSPIERTISKARGQAHQPSVYVLPPSREELSKNTVSLTCLIKDFFPPDIDVEWQSNGQQEPESKYRTTPPQLDEDGSYFLYSKLSVDKSRWQRGDTFICAVMHEALHNHYTQESLSHSPG

SEQ ID NO: 17 - protein, 225 aa, synthetic construct
  REGION 1..225: note = Canine IgGC Fc Fragment
CNNCPCPGCGLLGGPSVFIFPPKPKDILVTARTPTVTCVVVDLDPENPEVQISWFVDSKQVQTANTQPREEQSNGTYRVVSVLPIGHQDWLSGKQFKCKVNNKALPSPIEEIISKTPGQAHQPNVYVLPPSRDEMSKNTVTLTCLVKDFFPPEIDVEWQSNGQQEPESKYRMTPPQLDEDGSYFLYSKLSVDKSRWQRGDTFICAVMHEALHNHYTQISLSHSPG

SEQ ID NO: 18 - protein, 225 aa, synthetic construct
  REGION 1..225: note = Canine IgGD Fc Fragment
CISPCPVPESLGGPSVFIFPPKPKDILRITRTPEITCVVLDLGREDPEVQISWFVDGKEVHTAKTQPREQQFNSTYRVVSVLPIEHQDWLTGKEFKCRVNHIGLPSPIERTISKARGQAHQPSVYVLPPSPKELSSSDTVTLTCLIKDFFPPEIDVEWQSNGQPEPESKYHTTAPQLDEDGSYFLYSKLSVDKSRWQQGDTFTCAVMHEALQNHYTDLSLSHSPG

SEQ ID NO: 19 - protein, 224 aa, synthetic construct
  REGION 1..224: note = Feline IgG1a Fc Fragment
DCPKCPPPEMLGGPSIFIFPPKPKDTLSISRTPEVTCLVVDLGPDDSDVQITWFVDNTQVYTAKTSPREEQFNSTYRVVSVLPILHQDWLKGKEFKCKVNSKSLPSPIERTISKAKGQPHEPQVYVLPPAQEELSRNKVSVTCLIKSFHPPDIAVEWEITGQPEPENNYRTTPPQLDSDGTYFVYSKLSVDRSHWQRGNTYTCSVSHEALHSHHTQKSLTQSPG

SEQ ID NO: 20 - protein, 224 aa, synthetic construct
  REGION 1..224: note = Feline IgG1b Fc Fragment
DCPKCPPPEMLGGPSIFIFPPKPKDTLSISRTPEVTCLVVDLGPDDSDVQITWFVDNTQVYTAKTSPREEQFNSTYRVVSVLPILHQDWLKGKEFKCKVNSKSLPSPIERTISKDKGQPHEPQVYVLPPAQEELSRNKVSVTCLIEGFYPSDIAVEWEITGQPEPENNYRTTPPQLDSDGTYFLYSRLSVDRSRWQRGNTYTCSVSHEALHSHHTQKSLTQSPG

SEQ ID NO: 21 - protein, 225 aa, synthetic construct
  REGION 1..225: note = Feline IgG2 Fc Fragment
GEGPKCPVPEIPGAPSVFIFPPKPKDTLSISRTPEVTCLVVDLGPDDSNVQITWFVDNTEMHTAKTRPREEQFNSTYRVVSVLPILHQDWLKGKEFKCKVNSKSLPSAMERTISKAKGQPHEPQVYVLPPTQEELSENKVSVTCLIKGFHPPDIAVEWEITGQPEPENNYQTTPPQLDSDGTYFLYSRLSVDRSHWQRGNTYTCSVSHEALHSHHTQKSLTQSPG

SEQ ID NO: 22 - protein, 224 aa, synthetic construct
  REGION 1..224: note = Canine IgGB Fc Fragment with cNg-S Mutation
DCPKCPAPEMLGGPSVFIFPPKPKDTLLIARTPEVTCVVVDLDPEDPEVQISWFVDGKQMQTAKTQPREEQFSGTYRVVSVLPIGHQDWLKGKQFTCKVNNKALPSPIERTISKARGQAHQPSVYVLPPSREELSKNTVSLTCLIKDFFPPDIDVEWQSNGQQEPESKYRTTPPQLDEDGSYFLYSKLSVDKSRWQRGDTFICAVMHEALHNHYTQESLSHSPG

SEQ ID NO: 23 - protein, 224 aa, synthetic construct
  REGION 1..224: note = Feline IgG1b Fc Fragment with cNg-S Mutation
DCPKCPPPEMLGGPSIFIFPPKPKDTLSISRTPEVTCLVVDLGPDDSDVQITWFVDNTQVYTAKTSPREEQFSSTYRVVSVLPILHQDWLKGKEFKCKVNSKSLPSPIERTISKDKGQPHEPQVYVLPPAQEELSRNKVSVTCLIEGFYPSDIAVEWEITGQPEPENNYRTTPPQLDSDGTYFLYSRLSVDRSRWQRGNTYTCSVSHEALHSHHTQKSLTQSPG

SEQ ID NO: 24 - protein, 303 aa, synthetic construct
  REGION 1..303: note = Fusion Protein
  SITE 10: note = X is not D
  SITE 45: note = X is not H
  SITE 58: note = X is absent or N
FVNQHLCGSXLVEALELVCGERGFHYGGGGGGSGGGGGIVEQCCXSTCSLDQLENYCXGGGGGQGGGGQGGGGQGGGGGDCPKCPAPEMLGGPSVFIFPPKPKDTLLIARTPEVTCVVVDLDPEDPEVQISWFVDGKQMQTAKTQPREEQFNGTYRVVSVLPIGHQDWLKGKQFTCKVNNKALPSPIERTISKARGQAHQPSVYVLPPSREELSKNTVSLTCLIKDFFPPDIDVEWQSNGQQEPESKYRTTPPQLDEDGSYFLYSKLSVDKSRWQRGDTFICAVMHEALHNHYTQESLSHSPG

SEQ ID NO: 25 - protein, 303 aa, synthetic construct
  REGION 1..303: note = Fusion Protein
  SITE 58: note = X is absent or N
FVNQHLCGSHLVEALELVCGERGFHYGGGGGGSGGGGGIVEQCCTSTCSLDQLENYCXGGGGGQGGGGQGGGGQGGGGGDCPKCPAPEMLGGPSVFIFPPKPKDTLLIARTPEVTCVVVDLDPEDPEVQISWFVDGKQMQTAKTQPREEQFNGTYRVVSVLPIGHQDWLKGKQFTCKVNNKALPSPIERTISKARGQAHQPSVYVLPPSREELSKNTVSLTCLIKDFFPPDIDVEWQSNGQQEPESKYRTTPPQLDEDGSYFLYSKLSVDKSRWQRGDTFICAVMHEALHNHYTQESLSHSPG

SEQ ID NO: 26 - protein, 302 aa, synthetic construct
  REGION 1..302: note = Fusion Protein
  SITE 10: note = X is not D
  SITE 45: note = X is not H
FVNQHLCGSXLVEALALVCGERGFHYGGGGGGSGGGGGIVEQCCXSTCSLDQLENYCGGGGGQGGGGQGGGGQGGGGGDCPKCPAPEMLGGPSVFIFPPKPKDTLLIARTPEVTCVVVDLDPEDPEVQISWFVDGKQMQTAKTQPREEQFSGTYRVVSVLPIGHQDWLKGKQFTCKVNNKALPSPIERTISKARGQAHQPSVYVLPPSREELSKNTVSLTCLIKDFFPPDIDVEWQSNGQQEPESKYRTTPPQLDEDGSYFLYSKLSVDKSRWQRGDTFICAVMHEALHNHYTQESLSHSPG

SEQ ID NO: 27 - protein, 302 aa, synthetic construct
  REGION 1..302: note = Fusion Protein
  SITE 10: note = X is not D
  SITE 45: note = X is not H
FVNQHLCGSXLVEALELVCGERGFHYGGGGGGSGGGGGIVEQCCXSTCSLDQLENYCGGGGGQGGGGQGGGGQGGGGGDCPKCPPPEMLGGPSIFIFPPKPKDTLSISRTPEVTCLVVDLGPDDSDVQITWFVDNTQVYTAKTSPREEQFNSTYRVVSVLPILHQDWLKGKEFKCKVNSKSLPSPIERTISKDKGQPHEPQVYVLPPAQEELSRNKVSVTCLIEGFYPSDIAVEWEITGQPEPENNYRTTPPQLDSDGTYFLYSRLSVDRSRWQRGNTYTCSVSHEALHSHHTQKSLTQSPG

SEQ ID NO: 28 - protein, 302 aa, synthetic construct
  REGION 1..302: note = Fusion Protein
  SITE 10: note = X is not D
  SITE 45: note = X is not H
FVNQHLCGSXLVEALALVCGERGFHYGGGGGGSGGGGGIVEQCCXSTCSLDQLENYCGGGGGQGGGGQGGGGQGGGGGDCPKCPPPEMLGGPSIFIFPPKPKDTLSISRTPEVTCLVVDLGPDDSDVQITWFVDNTQVYTAKTSPREEQFSSTYRVVSVLPILHQDWLKGKEFKCKVNSKSLPSPIERTISKDKGQPHEPQVYVLPPAQEELSRNKVSVTCLIEGFYPSDIAVEWEITGQPEPENNYRTTPPQLDSDGTYFLYSRLSVDRSRWQRGNTYTCSVSHEALHSHHTQKSLTQSPG

SEQ ID NO: 29 - DNA, 57 bp, synthetic construct
  misc_feature 1..57: note = Leader DNA
  source 1..57: mol_type = other DNA
atggaatggagctgggtctttctcttcttcctgtcagtaacgactggtgtccactcc

SEQ ID NO: 30 - protein, 19 aa, synthetic construct
  REGION 1..19: note = Leader
MEWSWVFLFFLSVTTGVHS

SEQ ID NO: 31 - DNA, 966 bp, synthetic construct
  misc_feature 1..966: note = Fusion Protein DNA
  source 1..966: mol_type = other DNA
atggaatggagctgggtctttctcttcttcctgtcagtaacgactggtgtccactccttcgtgaaccagcacctgtgcggctcccacctggtggaagctctggaactcgtgtgcggcgagcggggcttccactacgggggtggcggaggaggttctggtggcggcggaggcatcgtggaacagtgctgcacctccacctgctccctggaccagctggaaaactactgcggtggcggaggtggtcaaggaggcggtggacagggtggaggtgggcagggaggaggcgggggagactgccccaagtgccccgctcccgagatgctgggcggacccagcgtgttcatcttccctcccaagcccaaggacacactgctgatcgccaggaccccggaggtgacctgcgtggtggtggacctggatcccgaagaccccgaggtgcagatcagctggttcgtggatggaaagcagatgcagaccgccaagacccaaccccgggaagagcagttcaacggcacctacagggtggtgagtgtgttgcccatcggccaccaggactggctgaaggggaagcaattcacatgcaaggttaataacaaggccctgcccagccccatcgagaggaccatcagcaaggccaggggccaggcccaccagccatctgtgtacgtgctgcccccatctagggaggaactgagcaagaacacagtcagccttacttgcctgatcaaggacttcttcccaccggacatagacgtggagtggcagagtaacggccagcaggagcccgagagcaagtataggaccacaccgccccaactggacgaggacggaagctacttcctctacagcaaattgagcgttgacaaaagcaggtggcagcgaggcgacaccttcatctgcgccgtgatgcacgaggctttgcataaccactacacccaggagagcctgtcccacagccccggatag

SEQ ID NO: 32 - protein, 302 aa, synthetic construct
  REGION 1..302: note = Fusion Protein
FVNQHLCGSHLVEALELVCGERGFHYGGGGGGSGGGGGIVEQCCTSTCSLDQLENYCGGGGGQGGGGQGGGGQGGGGGDCPKCPAPEMLGGPSVFIFPPKPKDTLLIARTPEVTCVVVDLDPEDPEVQISWFVDGKQMQTAKTQPREEQFNGTYRVVSVLPIGHQDWLKGKQFTCKVNNKALPSPIERTISKARGQAHQPSVYVLPPSREELSKNTVSLTCLIKDFFPPDIDVEWQSNGQQEPESKYRTTPPQLDEDGSYFLYSKLSVDKSRWQRGDTFICAVMHEALHNHYTQESLSHSPG

SEQ ID NO: 33 - DNA, 969 bp, synthetic construct
  misc_feature 1..969: note = Fusion Protein DNA
  source 1..969: mol_type = other DNA
atggaatggagctgggtctttctcttcttcctgtcagtaacgactggtgtccactccttcgtgaaccagcacctgtgcggctcccacctggtggaagctctggaactcgtgtgcggcgagcggggcttccactacgggggtggcggaggaggttctggtggcggcggaggcatcgtggaacagtgctgcacctccacctgctccctggaccagctggaaaactactgcaacggtggcggaggtggtcaaggaggcggtggacagggtggaggtgggcagggaggaggcgggggagactgccccaagtgccccgctcccgagatgctgggcggacccagcgtgttcatcttccctcccaagcccaaggacacactgctgatcgccaggaccccggaggtgacctgcgtggtggtggacctggatcccgaagaccccgaggtgcagatcagctggttcgtggatggaaagcagatgcagaccgccaagacccaaccccgggaagagcagttcaacggcacctacagggtggtgagtgtgttgcccatcggccaccaggactggctgaaggggaagcaattcacatgcaaggttaataacaaggccctgcccagccccatcgagaggaccatcagcaaggccaggggccaggcccaccagccatctgtgtacgtgctgcccccatctagggaggaactgagcaagaacacagtcagccttacttgcctgatcaaggacttcttcccaccggacatagacgtggagtggcagagtaacggccagcaggagcccgagagcaagtataggaccacaccgccccaactggacgaggacggaagctacttcctctacagcaaattgagcgttgacaaaagcaggtggcagcgaggcgacaccttcatctgcgccgtgatgcacgaggctttgcataaccactacacccaggagagcctgtcccacagccccggatag

SEQ ID NO: 34 - protein, 303 aa, synthetic construct
  REGION 1..303: note = Fusion Protein
FVNQHLCGSHLVEALELVCGERGFHYGGGGGGSGGGGGIVEQCCTSTCSLDQLENYCNGGGGGQGGGGQGGGGQGGGGGDCPKCPAPEMLGGPSVFIFPPKPKDTLLIARTPEVTCVVVDLDPEDPEVQISWFVDGKQMQTAKTQPREEQFNGTYRVVSVLPIGHQDWLKGKQFTCKVNNKALPSPIERTISKARGQAHQPSVYVLPPSREELSKNTVSLTCLIKDFFPPDIDVEWQSNGQQEPESKYRTTPPQLDEDGSYFLYSKLSVDKSRWQRGDTFICAVMHEALHNHYTQESLSHSPG

SEQ ID NO: 35 - DNA, 966 bp, synthetic construct
  misc_feature 1..966: note = Fusion Protein DNA
  source 1..966: mol_type = other DNA
atggaatggagctgggtctttctcttcttcctgtcagtaacgactggtgtccactccttcgtgaaccagcacctgtgcggctcccacctggtggaagctctggcactcgtgtgcggcgagcggggcttccactacgggggtggcggaggaggttctggtggcggcggaggcatcgtggaacagtgctgcacctccacctgctccctggaccagctggaaaactactgcggtggcggaggtggtcaaggaggcggtggacagggtggaggtgggcagggaggaggcgggggagactgccccaagtgccccgctcccgagatgctgggcggacccagcgtgttcatcttccctcccaagcccaaggacacactgctgatcgccaggaccccggaggtgacctgcgtggtggtggacctggatcccgaagaccccgaggtgcagatcagctggttcgtggatggaaagcagatgcagaccgccaagacccaaccccgggaagagcagttctcaggcacctacagggtggtgagtgtgttgcccatcggccaccaggactggctgaaggggaagcaattcacatgcaaggttaataacaaggccctgcccagccccatcgagaggaccatcagcaaggccaggggccaggcccaccagccatctgtgtacgtgctgcccccatctagggaggaactgagcaagaacacagtcagccttacttgcctgatcaaggacttcttcccaccggacatagacgtggagtggcagagtaacggccagcaggagcccgagagcaagtataggaccacaccgccccaactggacgaggacggaagctacttcctctacagcaaattgagcgttgacaaaagcaggtggcagcgaggcgacaccttcatctgcgccgtgatgcacgaggctttgcataaccactacacccaggagagcctgtcccacagccccggatag

SEQ ID NO: 36 - protein, 302 aa, synthetic construct
  REGION 1..302: note = Fusion Protein
FVNQHLCGSHLVEALALVCGERGFHYGGGGGGSGGGGGIVEQCCTSTCSLDQLENYCGGGGGQGGGGQGGGGQGGGGGDCPKCPAPEMLGGPSVFIFPPKPKDTLLIARTPEVTCVVVDLDPEDPEVQISWFVDGKQMQTAKTQPREEQFSGTYRVVSVLPIGHQDWLKGKQFTCKVNNKALPSPIERTISKARGQAHQPSVYVLPPSREELSKNTVSLTCLIKDFFPPDIDVEWQSNGQQEPESKYRTTPPQLDEDGSYFLYSKLSVDKSRWQRGDTFICAVMHEALHNHYTQESLSHSPG

SEQ ID NO: 37 - DNA, 966 bp, synthetic construct
  misc_feature 1..966: note = Fusion Protein DNA
  source 1..966: mol_type = other DNA
atggaatggagctgggtctttctcttcttcctgtcagtaacgactggtgtccactccttcgtgaaccagcacctgtgcggctcccacctggtggaagctctggaactcgtgtgcggcgagcggggcttccactacgggggtggcggaggaggttctggtggcggcggaggcatcgtggaacagtgctgcacctccacctgctccctggaccagctggaaaactactgcggtggcggaggtggtcaaggaggcggtggacagggtggaggtgggcagggaggaggcgggggagactgccccaaatgtcctccgcctgagatgctgggtggccctagcatcttcatcttcccgcccaagcccaaggatactctgtccattagcaggacccccgaggtgacctgcctggtggtggacctggggccagacgactctgacgtgcagatcacctggttcgtagacaacacccaggtttacactgccaagaccagtcccagggaggagcagttcaacagcacatacagggtggtgagcgttctgcccatcctgcaccaggactggctgaaaggcaaagagttcaagtgtaaggtgaacagcaagagcctgcccagccccattgaaaggaccatcagcaaggacaagggccagccgcacgagccccaagtctacgtgctgcccccagcacaggaagagctgagcaggaacaaggttagcgtgacatgcctgatcgagggtttctaccccagcgacatcgccgtggagtgggaaatcaccggccaacccgagcccgagaacaactacaggaccactccgccgcaactggacagcgacgggacctacttcttgtatagcaggctgagcgtggaccggagcaggtggcagaggggcaacacctacacttgcagcgtgagccacgaggccttgcacagccaccacactcagaagagtctgacccagagcccgggatag

SEQ ID NO: 38 - protein, 302 aa, synthetic construct
  REGION 1..302: note = Fusion Protein
FVNQHLCGSHLVEALELVCGERGFHYGGGGGGSGGGGGIVEQCCTSTCSLDQLENYCGGGGGQGGGGQGGGGQGGGGGDCPKCPPPEMLGGPSIFIFPPKPKDTLSISRTPEVTCLVVDLGPDDSDVQITWFVDNTQVYTAKTSPREEQFNSTYRVVSVLPILHQDWLKGKEFKCKVNSKSLPSPIERTISKDKGQPHEPQVYVLPPAQEELSRNKVSVTCLIEGFYPSDIAVEWEITGQPEPENNYRTTPPQLDSDGTYFLYSRLSVDRSRWQRGNTYTCSVSHEALHSHHTQKSLTQSPG

SEQ ID NO: 39 - DNA, 966 bp, synthetic construct
  misc_feature 1..966: note = Fusion Protein DNA
  source 1..966: mol_type = other DNA
atggaatggagctgggtctttctcttcttcctgtcagtaacgactggtgtccactccttcgtgaaccagcacctgtgcggctcccacctggtggaagctctggcactcgtgtgcggcgagcggggcttccactacgggggtggcggaggaggttctggtggcggcggaggcatcgtggaacagtgctgcacctccacctgctccctggaccagctggaaaactactgcggtggcggaggtggtcaaggaggcggtggacagggtggaggtgggcagggaggaggcgggggagactgccccaaatgtcctccgcctgagatgctgggtggccctagcatcttcatcttcccgcccaagcccaaggatactctgtccattagcaggacccccgaggtgacctgcctggtggtggacctggggccagacgactctgacgtgcagatcacctggttcgtagacaacacccaggtttacactgccaagaccagtcccagggaggagcagttcagcagcacatacagggtggtgagcgttctgcccatcctgcaccaggactggctgaaaggcaaagagttcaagtgtaaggtgaacagcaagagcctgcccagccccattgaaaggaccatcagcaaggacaagggccagccgcacgagccccaagtctacgtgctgcccccagcacaggaagagctgagcaggaacaaggttagcgtgacatgcctgatcgagggtttctaccccagcgacatcgccgtggagtgggaaatcaccggccaacccgagcccgagaacaactacaggaccactccgccgcaactggacagcgacgggacctacttcttgtatagcaggctgagcgtggaccggagcaggtggcagaggggcaacacctacacttgcagcgtgagccacgaggccttgcacagccaccacactcagaagagtctgacccagagcccgggatag

SEQ ID NO: 40 - protein, 302 aa, synthetic construct
  REGION 1..302: note = Fusion Protein
FVNQHLCGSHLVEALALVCGERGFHYGGGGGGSGGGGGIVEQCCTSTCSLDQLENYCGGGGGQGGGGQGGGGQGGGGGDCPKCPPPEMLGGPSIFIFPPKPKDTLSISRTPEVTCLVVDLGPDDSDVQITWFVDNTQVYTAKTSPREEQFSSTYRVVSVLPILHQDWLKGKEFKCKVNSKSLPSPIERTISKDKGQPHEPQVYVLPPAQEELSRNKVSVTCLIEGFYPSDIAVEWEITGQPEPENNYRTTPPQLDSDGTYFLYSRLSVDRSRWQRGNTYTCSVSHEALHSHHTQKSLTQSPG

SEQ ID NO: 41 - DNA, 942 bp, synthetic construct
  misc_feature 1..942: note = Fusion Protein DNA
  source 1..942: mol_type = other DNA
atggaatggagctgggtctttctcttcttcctgtcagtaacgactggtgtccactccttcgtgaaccagcacctgtgcggctccgacctggtggaagctctggctctcgtgtgcggcgagcggggcttcttctacaccgatcccactggaggcggtccacgcagaggcatcgtggaacagtgctgccactccatctgctccctgtaccagctggaaaactactgcaatggcggaggtggtgcaggaggcggtggacgctgcactgacacccctccatgccctgtgcccgagcccctgggtggccccagcgtactgatcttcccaccgaaacccaaggacatcctgaggatcacccgcaccccggaggtgacctgcgtggtgctggacctgggcagggaggaccccgaagtgcaaatcagctggttcgtggacggaaaggaggtgcacaccgccaagacccaatcaagggagcagcagttcaacggcacctacagggtggtgagcgtgttgcccatagagcaccaggactggctgaccggcaaggagttcaagtgccgcgtgaaccacattgatctccccagccccatcgagaggactatctccaaggcccgagggagggcccacaagcccagtgtatacgtgctgccgccctctccgaaggaactgagctctagcgacaccgtgagcatcacctgcctgatcaaggacttctaccctcccgacatagacgtagagtggcagagcaacggccagcaggagcccgaaaggaagcacaggatgaccccaccccaactggacgaggacggctcatactttctttatagcaagctgagtgtggacaagagcaggtggcagcagggcgaccctttcacttgcgccgtaatgcacgagaccctgcagaatcactacaccgacctgtcactgagccatagccccggatag

SEQ ID NO: 42 - protein, 294 aa, synthetic construct
  REGION 1..294: note = Fusion Protein
FVNQHLCGSDLVEALALVCGERGFFYTDPTGGGPRRGIVEQCCHSICSLYQLENYCNGGGGAGGGGRCTDTPPCPVPEPLGGPSVLIFPPKPKDILRITRTPEVTCVVLDLGREDPEVQISWFVDGKEVHTAKTQSREQQFNGTYRVVSVLPIEHQDWLTGKEFKCRVNHIDLPSPIERTISKARGRAHKPSVYVLPPSPKELSSSDTVSITCLIKDFYPPDIDVEWQSNGQQEPERKHRMTPPQLDEDGSYFLYSKLSVDKSRWQQGDPFTCAVMHETLQNHYTDLSLSHSPG

SEQ ID NO: 43 - DNA, 942 bp, synthetic construct
  misc_feature 1..942: note = Fusion Protein DNA
  source 1..942: mol_type = other DNA
atggaatggagctgggtctttctcttcttcctgtcagtaacgactggtgtccactccttcgtgaaccagcacctgtgcggctccgacctggtggaagctctggctctcgtgtgcggcgagcggggcttcttctacaccgatcccactggaggcggtccacgcagaggcatcgtggaacagtgctgccactccatctgctccctgtaccagctggaaaactactgcaatggcggaggtggtgcaggaggcggtggacgctgcactgacacccctccatgccctgtgcccgagcccctgggtggccccagcgtactgatcttcccaccgaaacccaaggacatcctgaggatcacccgcaccccggaggtgacctgcgtggtgctggacctgggcagggaggaccccgaagtgcaaatcagctggttcgtggacggaaaggaggtgcacaccgccaagacccaatcaagggagcagcagttcaacggcacctacagggtggtgagcgtgttgcccatagagcaccaggactggctgaccggcaaggagttcaagtgccgcgtgaaccacattgatctccccagccccatcgagaggactatctccaaggcccgagggagggcccacaagcccagtgtatacgtgctgccgccctctccgaaggaactgagctctagcgacaccgtgagcatcacctgcctgatcaaggacttctaccctcccgacatagacgtagagtggcagagcaacggccagcaggagcccgaaaggaagcacaggatgaccccaccccaactggacgaggacggctcatactttctttatagcaagctgagtgtggacaagagcaggtggcagcagggcgaccctttcacttgcgccgtactgcacgaggccctgcactctcactacacccagaagtcactgagccttagccccggatag

SEQ ID NO: 44 - protein, 294 aa, synthetic construct
  REGION 1..294: note = Fusion Protein
FVNQHLCGSDLVEALALVCGERGFFYTDPTGGGPRRGIVEQCCHSICSLYQLENYCNGGGGAGGGGRCTDTPPCPVPEPLGGPSVLIFPPKPKDILRITRTPEVTCVVLDLGREDPEVQISWFVDGKEVHTAKTQSREQQFNGTYRVVSVLPIEHQDWLTGKEFKCRVNHIDLPSPIERTISKARGRAHKPSVYVLPPSPKELSSSDTVSITCLIKDFYPPDIDVEWQSNGQQEPERKHRMTPPQLDEDGSYFLYSKLSVDKSRWQQGDPFTCAVLHEALHSHYTQKSLSLSPG

SEQ ID NO: 45 - DNA, 942 bp, synthetic construct
  misc_feature 1..942: note = Fusion Protein DNA
  source 1..942: mol_type = other DNA
atggaatggagctgggtctttctcttcttcctgtcagtaacgactggtgtccactccttcgtgaaccagcacctgtgcggctccgacctggtggaagctctggctctcgtgtgcggcgagcggggcttcttctacaccgatcccactggaggcggtccacgcagaggcatcgtggaacagtgctgccactccatctgctccctgtaccagctggaaaactactgcaatggcggaggtggtgcaggaggcggtggacgctgcactgacacccctccatgccctgtgcccgagcccctgggtggccccagcgtactgatcttcccaccgaaacccaaggacatcctgaggatcacccgcaccccggaggtgacctgcgtggtgctggacctgggcagggaggaccccgaagtgcaaatcagctggttcgtggacggaaaggaggtgcacaccgccaagacccaatcaagggagcagcagttcaacggcacctacagggtggtgagcgtgttgcccatagagcaccaggactggctgaccggcaaggagttcaagtgccgcgtgaaccacattgatctccccagccccatcgagaggactatctccaaggcccgagggagggcccacaagcccagtgtatacgtgctgccgccctctccgaaggaactgagctctagcgacaccgtgagcatcacctgcctgatcaaggacttctaccctcccgacatagacgtagagtggcagagcaacggccagcaggagcccgaaaggaagcacaggatgaccccaccccaactggacgaggacggctcatactttctttatagcaagctgagtgtggacaagagcaggtggcagcagggcgaccctttcacttgcgccgtactgcacgagaccctgcagtctcactacaccgacctgtcactgagccatagccccggatag

SEQ ID NO: 46 - protein, 294 aa, synthetic construct
  REGION 1..294: note = Fusion Protein
FVNQHLCGSDLVEALALVCGERGFFYTDPTGGGPRRGIVEQCCHSICSLYQLENYCNGGGGAGGGGRCTDTPPCPVPEPLGGPSVLIFPPKPKDILRITRTPEVTCVVLDLGREDPEVQISWFVDGKEVHTAKTQSREQQFNGTYRVVSVLPIEHQDWLTGKEFKCRVNHIDLPSPIERTISKARGRAHKPSVYVLPPSPKELSSSDTVSITCLIKDFYPPDIDVEWQSNGQQEPERKHRMTPPQLDEDGSYFLYSKLSVDKSRWQQGDPFTCAVLHETLQSHYTDLSLSHSPG

SEQ ID NO: 47 - DNA, 942 bp, synthetic construct
  misc_feature 1..942: note = Fusion Protein DNA
  source 1..942: mol_type = other DNA
atggaatggagctgggtctttctcttcttcctgtcagtaacgactggtgtccactccttcgtgaaccagcacctgtgcggctccgacctggtggaagctctggctctcgtgtgcggcgagcggggcttcttctacaccgatcccactggaggcggtccacgcagaggcatcgtggaacagtgctgccactccatctgctccctgtaccagctggaaaactactgcaatggcggaggtggtgcaggaggcggtggacgctgcactgacacccctccatgccctgtgcccgagcccctgggtggccccagcgtactgatcttcccaccgaaacccaaggacatcctgaggatcacccgcaccccggaggtgacctgcgtggtgctggacctgggcagggaggaccccgaagtgcaaatcagctggttcgtggacggaaaggaggtgcacaccgccaagacccaatcaagggagcagcagttcaacggcacctacagggtggtgagcgtgttgcccatagagcaccaggactggctgaccggcaaggagttcaagtgccgcgtgaaccacattgatctccccagccccatcgagaggactatctccaaggcccgagggagggcccacaagcccagtgtatacgtgctgccgccctctccgaaggaactgagctctagcgacaccgtgagcatcacctgcctgatcaaggacttctaccctcccgacatagacgtagagtggcagagcaacggccagcaggagcccgaaaggaagcacaggatgaccccaccccaactggacgaggacggctcatactttctttatagcaagctgagtgtggacaagagcaggtggcagcagggcgaccctttcacttgcgccgtaatgcacgagaccctgcagtctcactacaccgacctgtcactgagccatagccccggatag

SEQ ID NO: 48 - protein, 294 aa, synthetic construct
  REGION 1..294: note = Fusion Protein
FVNQHLCGSDLVEALALVCGERGFFYTDPTGGGPRRGIVEQCCHSICSLYQLENYCNGGGGAGGGGRCTDTPPCPVPEPLGGPSVLIFPPKPKDILRITRTPEVTCVVLDLGREDPEVQISWFVDGKEVHTAKTQSREQQFNGTYRVVSVLPIEHQDWLTGKEFKCRVNHIDLPSPIERTISKARGRAHKPSVYVLPPSPKELSSSDTVSITCLIKDFYPPDIDVEWQSNGQQEPERKHRMTPPQLDEDGSYFLYSKLSVDKSRWQQGDPFTCAVMHETLQSHYTDLSLSHSPG

SEQ ID NO: 49 - DNA, 942 bp, synthetic construct
  misc_feature 1..942: note = Fusion Protein DNA
  source 1..942: mol_type = other DNA
atggaatggagctgggtctttctcttcttcctgtcagtaacgactggtgtccactccttcgtgaaccagcacctgtgcggctccgacctggtggaagctctggctctcgtgtgcggcgagcggggcttcttctacaccgatcccactggaggcggtccacgcagaggcatcgtggaacagtgctgccactccatctgctccctgtaccagctggaaaactactgcaatggcggaggtggtgcaggaggcggtggacgctgcactgacacccctccatgccctgtgcccgagcccctgggtggccccagcgtactgatcttcccaccgaaacccaaggacatcctgaggatcacccgcaccccggaggtgacctgcgtggtgctggacctgggcagggaggaccccgaagtgcaaatcagctggttcgtggacggaaaggaggtgcacaccgccaagacccaatcaagggagcagcagttcaacggcacctacagggtggtgagcgtgttgcccatagagcaccaggactggctgaccggcaaggagttcaagtgccgcgtgaaccacattgatctccccagccccatcgagaggactatctccaaggcccgagggagggcccacaagcccagtgtatacgtgctgccgccctctccgaaggaactgagctctagcgacaccgtgagcatcacctgcctgatcaaggacttctaccctcccgacatagacgtagagtggcagagcaacggccagcaggagcccgaaaggaagcacaggatgaccccaccccaactggacgaggacggctcatactttctttatagcaagctgagtgtggacaagagcaggtggcagcagggcgaccctttcacttgcgccgtactgcacgagaccctgcagaatcactacaccgacctgtcactgagccatagccccggatag

SEQ ID NO: 50 - protein, 294 aa, synthetic construct
  REGION 1..294: note = Fusion Protein
FVNQHLCGSDLVEALALVCGERGFFYTDPTGGGPRRGIVEQCCHSICSLYQLENYCNGGGGAGGGGRCTDTPPCPVPEPLGGPSVLIFPPKPKDILRITRTPEVTCVVLDLGREDPEVQISWFVDGKEVHTAKTQSREQQFNGTYRVVSVLPIEHQDWLTGKEFKCRVNHIDLPSPIERTISKARGRAHKPSVYVLPPSPKELSSSDTVSITCLIKDFYPPDIDVEWQSNGQQEPERKHRMTPPQLDEDGSYFLYSKLSVDKSRWQQGDPFTCAVLHETLQNHYTDLSLSHSPG

SEQ ID NO: 51 - DNA, 930 bp, synthetic construct
  misc_feature 1..930: note = Fusion Protein DNA
  source 1..930: mol_type = other DNA
atggaatggagctgggtctttctcttcttcctgtcagtaacgactggtgtccactccttcgtgaaccagcacctgtgcggctccgacctggtggaagctctggctctcgtgtgcggcgagcggggcttcttctacaccgatcccactggaggcggtccacgcagaggcatcgtggaacagtgctgccactccatctgctccctgtaccagctggaaaactactgcaatggcggaggtggtgcaggaggcggtggagactgccccaagtgccccgctcccgagatgctgggcggacccagcgtgttcatcttccctcccaagcccaaggacacactgctgatcgccaggaccccggaggtgacctgcgtggtggtggacctggatcccgaagaccccgaggtgcagatcagctggttcgtggatggaaagcagatgcagaccgccaagacccaaccccgggaagagcagttcaacggcacctacagggtggtgagtgtgttgcccatcggccaccaggactggctgaaggggaagcaattcacatgcaaggttaataacaaggccctgcccagccccatcgagaggaccatcagcaaggccaggggccaggcccaccagccatctgtgtacgtgctgcccccatctagggaggaactgagcaagaacacagtcagccttacttgcctgatcaaggacttcttcccaccggacatagacgtggagtggcagagtaacggccagcaggagcccgagagcaagtataggaccacaccgccccaactggacgaggacggaagctacttcctctacagcaaattgagcgttgacaaaagcaggtggcagcgaggcgacaccttcatctgcgccgtgatgcacgaggctttgcataaccactacacccaggagagcctgtcccacagccccggatag

SEQ ID NO: 52 - protein, 290 aa, synthetic construct
  REGION 1..290: note = Fusion Protein
FVNQHLCGSDLVEALALVCGERGFFYTDPTGGGPRRGIVEQCCHSICSLYQLENYCNGGGGAGGGGDCPKCPAPEMLGGPSVFIFPPKPKDTLLIARTPEVTCVVVDLDPEDPEVQISWFVDGKQMQTAKTQPREEQFNGTYRVVSVLPIGHQDWLKGKQFTCKVNNKALPSPIERTISKARGQAHQPSVYVLPPSREELSKNTVSLTCLIKDFFPPDIDVEWQSNGQQEPESKYRTTPPQLDEDGSYFLYSKLSVDKSRWQRGDTFICAVMHEALHNHYTQESLSHSPG

SEQ ID NO: 53 - DNA, 933 bp, synthetic construct
  misc_feature 1..933: note = Fusion Protein DNA
  source 1..933: mol_type = other DNA
atggaatggagctgggtctttctcttcttcctgtcagtaacgactggtgtccactccttcgtgaaccagcacctgtgcggctccgacctggtggaagctctggctctcgtgtgcggcgagcggggcttcttctacaccgatcccactggaggcggtccacgcagaggcatcgtggaacagtgctgccactccatctgctccctgtaccagctggaaaactactgcaatggcggaggtggtgcaggaggcggtggatgcaacaactgcccgtgtccgggatgcggcctcctgggcggaccgagcgtgttcattttccctcctaagcccaaggacattctggtgaccgccaggacccccacggtgacctgcgtggtagtagatctcgatcccgaaaacccagaggtgcaaatcagctggttcgtggactctaagcaagtgcaaaccgccaacacgcaaccccgcgaggaacagagcaacggcacctacagggtggtgagcgtgctgcccatcgggcatcaggactggctgagcggcaagcagtttaaatgcaaggttaacaacaaggcactgcccagccccatcgaggagatcatcagcaagaccccgggacaggcccaccagcccaacgtgtacgtccttcctccgagccgcgacgagatgagcaagaacaccgtgacgctgacctgtttggtgaaggacttcttcccacccgagatcgacgtggagtggcaaagcaatggccagcaggagcccgagagcaaatacaggatgaccccaccccaactggatgaggatggcagctatttcctctacagcaaattgtccgtggacaaaagcaggtggcagaggggcgacaccttcatctgcgccgtcatgcacgaggcccttcacaatcactacacccagatcagcctgagccactctcccggatag

SEQ ID NO: 54 - protein, 291 aa, synthetic construct
  REGION 1..291: note = Fusion Protein
FVNQHLCGSDLVEALALVCGERGFFYTDPTGGGPRRGIVEQCCHSICSLYQLENYCNGGGGAGGGGCNNCPCPGCGLLGGPSVFIFPPKPKDILVTARTPTVTCVVVDLDPENPEVQISWFVDSKQVQTANTQPREEQSNGTYRVVSVLPIGHQDWLSGKQFKCKVNNKALPSPIEEIISKTPGQAHQPNVYVLPPSRDEMSKNTVTLTCLVKDFFPPEIDVEWQSNGQQEPESKYRMTPPQLDEDGSYFLYSKLSVDKSRWQRGDTFICAVMHEALHNHYTQISLSHSPG

SEQ ID NO: 55 - DNA, 933 bp, synthetic construct
  misc_feature 1..933: note = Fusion Protein DNA
  source 1..933: mol_type = other DNA
atggaatggagctgggtctttctcttcttcctgtcagtaacgactggtgtccactccttcgtgaaccagcacctgtgcggctccgacctggtggaagctctggctctcgtgtgcggcgagcggggcttcttctacaccgatcccactggaggcggtccacgcagaggcatcgtggaacagtgctgccactccatctgctccctgtaccagctggaaaactactgcaatggcggaggtggtgcaggaggcggtggatgcatcagcccctgccccgtgccggagagcctgggtggccctagcgtgttcatattccctcccaagcccaaggacatcctgaggatcaccaggacccccgagatcacctgtgtggtgctggatcttggcagggaagaccccgaagtccagatcagctggttcgtggatggcaaggaggtgcacaccgccaagacccagccgagggagcagcagttcaactccacctacagggtggtgagcgtgctgcctatcgagcatcaggactggctgaccggcaaagagttcaagtgcagggtgaaccacatcggcctgcccagccccatcgagaggaccatcagcaaagccaggggccaggcccaccagcccagtgtgtacgtgcttccccctagcccaaaggaactgagtagcagcgataccgtgaccctgacctgcctgatcaaggactttttcccgccagaaatagacgtggagtggcagagcaacggccagccggagcccgagagcaaataccacaccaccgcccctcaactggacgaggacgggagctacttcctgtatagcaagctgagcgttgacaagagcaggtggcaacagggcgacaccttcacctgcgccgtgatgcacgaagctctgcaaaaccactacaccgacctgtcactgagccatagccccggatag

SEQ ID NO: 56 - protein, 291 aa, synthetic construct
  REGION 1..291: note = Fusion Protein
FVNQHLCGSDLVEALALVCGERGFFYTDPTGGGPRRGIVEQCCHSICSLYQLENYCNGGGGAGGGGCISPCPVPESLGGPSVFIFPPKPKDILRITRTPEITCVVLDLGREDPEVQISWFVDGKEVHTAKTQPREQQFNSTYRVVSVLPIEHQDWLTGKEFKCRVNHIGLPSPIERTISKARGQAHQPSVYVLPPSPKELSSSDTVTLTCLIKDFFPPEIDVEWQSNGQPEPESKYHTTAPQLDEDGSYFLYSKLSVDKSRWQQGDTFTCAVMHEALQNHYTDLSLSHSPG

SEQ ID NO: 57 - DNA, 930 bp, synthetic construct
  misc_feature 1..930: note = Fusion Protein DNA
  source 1..930: mol_type = other DNA
atggaatggagctgggtctttctcttcttcctgtcagtaacgactggtgtccactccttcgtgaaccagcacctgtgcggctccgacctggtggaagctctggctctcgtgtgcggcgagcggggcttcttctacaccgatcccactggaggcggtccacgcagaggcatcgtggaacagtgctgccactccatctgctccctgtaccagctggaaaactactgcaatggcggaggtggtgcaggaggcggtggagactgccccaagtgccccgctcccgagatgctgggcggacccagcgtgttcatcttccctcccaagcccaaggacacactgctgatcgccaggaccccggaggtgacctgcgtggtggtggacctggatcccgaagaccccgaggtgcagatcagctggttcgtggatggaaagcagatgcagaccgccaagacccaaccccgggaagagcagttccaaggcacctacagggtggtgagtgtgttgcccatcggccaccaggactggctgaaggggaagcaattcacatgcaaggttaataacaaggccctgcccagccccatcgagaggaccatcagcaaggccaggggccaggcccaccagccatctgtgtacgtgctgcccccatctagggaggaactgagcaagaacacagtcagccttacttgcctgatcaaggacttcttcccaccggacatagacgtggagtggcagagtaacggccagcaggagcccgagagcaagtataggaccacaccgccccaactggacgaggacggaagctacttcctctacagcaaattgagcgttgacaaaagcaggtggcagcgaggcgacaccttcatctgcgccgtgatgcacgaggctttgcataaccactacacccaggagagcctgtcccacagccccggatag

SEQ ID NO: 58 - protein, 290 aa, synthetic construct
  REGION 1..290: note = Fusion Protein
FVNQHLCGSDLVEALALVCGERGFFYTDPTGGGPRRGIVEQCCHSICSLYQLENYCNGGGGAGGGGDCPKCPAPEMLGGPSVFIFPPKPKDTLLIARTPEVTCVVVDLDPEDPEVQISWFVDGKQMQTAKTQPREEQFQGTYRVVSVLPIGHQDWLKGKQFTCKVNNKALPSPIERTISKARGQAHQPSVYVLPPSREELSKNTVSLTCLIKDFFPPDIDVEWQSNGQQEPESKYRTTPPQLDEDGSYFLYSKLSVDKSRWQRGDTFICAVMHEALHNHYTQESLSHSPG

SEQ ID NO: 59 - DNA, 930 bp, synthetic construct
  misc_feature 1..930: note = Fusion Protein DNA
  source 1..930: mol_type = other DNA
atggaatggagctgggtctttctcttcttcctgtcagtaacgactggtgtccactccttcgtgaaccagcacctgtgcggctccgacctggtggaagctctggctctcgtgtgcggcgagcggggcttcttctacaccgatcccactggaggcggtccacgcagaggcatcgtggaacagtgctgccactccatctgctccctgtaccagctggaaaactactgcaatggcggaggtggtgcaggaggcggtggagactgccccaagtgccccgctcccgagatgctgggcggacccagcgtgttcatcttccctcccaagcccaaggacacactgctgatcgccaggaccccggaggtgacctgcgtggtggtggacctggatcccgaagaccccgaggtgcagatcagctggttcgtggatggaaagcagatgcagaccgccaagacccaaccccgggaagagcagttcagcggcacctacagggtggtgagtgtgttgcccatcggccaccaggactggctgaaggggaagcaattcacatgcaaggttaataacaaggccctgcccagccccatcgagaggaccatcagcaaggccaggggccaggcccaccagccatctgtgtacgtgctgcccccatctagggaggaactgagcaagaacacagtcagccttacttgcctgatcaaggacttcttcccaccggacatagacgtggagtggcagagtaacggccagcaggagcccgagagcaagtataggaccacaccgccccaactggacgaggacggaagctacttcctctacagcaaattgagcgttgacaaaagcaggtggcagcgaggcgacaccttcatctgcgccgtgatgcacgaggctttgcataaccactacacccaggagagcctgtcccacagccccggatag

SEQ ID NO: 60 - protein, 290 aa, synthetic construct
  REGION 1..290: note = Fusion Protein
FVNQHLCGSDLVEALALVCGERGFFYTDPTGGGPRRGIVEQCCHSICSLYQLENYCNGGGGAGGGGDCPKCPAPEMLGGPSVFIFPPKPKDTLLIARTPEVTCVVVDLDPEDPEVQISWFVDGKQMQTAKTQPREEQFSGTYRVVSVLPIGHQDWLKGKQFTCKVNNKALPSPIERTISKARGQAHQPSVYVLPPSREELSKNTVSLTCLIKDFFPPDIDVEWQSNGQQEPESKYRTTPPQLDEDGSYFLYSKLSVDKSRWQRGDTFICAVMHEALHNHYTQESLSHSPG

SEQ ID NO: 61 - DNA, 930 bp, synthetic construct
  misc_feature 1..930: note = Fusion Protein DNA
  source 1..930: mol_type = other DNA
atggaatggagctgggtctttctcttcttcctgtcagtaacgactggtgtccactccttcgtgaaccagcacctgtgcggctccgacctggtggaagctctggctctcgtgtgcggcgagcggggcttcttctacaccgatcccactggaggcggtccacgcagaggcatcgtggaacagtgctgccactccatctgctccctgtaccagctggaaaactactgcaatggcggaggtggtgcaggaggcggtggagactgccccaagtgccccgctcccgagatgctgggcggacccagcgtgttcatcttccctcccaagcccaaggacacactgctgatcgccaggaccccggaggtgacctgcgtggtggtggacctggatcccgaagaccccgaggtgcagatcagctggttcgtggatggaaagcagatgcagaccgccaagacccaaccccgggaagagcagttcgacggcacctacagggtggtgagtgtgttgcccatcggccaccaggactggctgaaggggaagcaattcacatgcaaggttaataacaaggccctgcccagccccatcgagaggaccatcagcaaggccaggggccaggcccaccagccatctgtgtacgtgctgcccccatctagggaggaactgagcaagaacacagtcagccttacttgcctgatcaaggacttcttcccaccggacatagacgtggagtggcagagtaacggccagcaggagcccgagagcaagtataggaccacaccgccccaactggacgaggacggaagctacttcctctacagcaaattgagcgttgacaaaagcaggtggcagcgaggcgacaccttcatctgcgccgtgatgcacgaggctttgcataaccactacacccaggagagcctgtcccacagccccggatag

SEQ ID NO: 62 - protein, 290 aa, synthetic construct
  REGION 1..290: note = Fusion Protein
FVNQHLCGSDLVEALALVCGERGFFYTDPTGGGPRRGIVEQCCHSICSLYQLENYCNGGGGAGGGGDCPKCPAPEMLGGPSVFIFPPKPKDTLLIARTPEVTCVVVDLDPEDPEVQISWFVDGKQMQTAKTQPREEQFDGTYRVVSVLPIGHQDWLKGKQFTCKVNNKALPSPIERTISKARGQAHQPSVYVLPPSREELSKNTVSLTCLIKDFFPPDIDVEWQSNGQQEPESKYRTTPPQLDEDGSYFLYSKLSVDKSRWQRGDTFICAVMHEALHNHYTQESLSHSPG

SEQ ID NO: 63 - DNA, 930 bp, synthetic construct
  misc_feature 1..930: note = Fusion Protein DNA
  source 1..930: mol_type = other DNA
atggaatggagctgggtctttctcttcttcctgtcagtaacgactggtgtccactccttcgtgaaccagcacctgtgcggctccgacctggtggaagctctggctctcgtgtgcggcgagcggggcttcttctacaccgatcccactggaggcggtccacgcagaggcatcgtggaacagtgctgccactccatctgctccctgtaccagctggaaaactactgcaatggcggaggtggtgcaggaggcggtggagactgccccaagtgccccgctcccgagatgctgggcggacccagcgtgttcatcttccctcccaagcccaaggacacactgctgatcgccaggaccccggaggtgacctgcgtggtggtggacctggatcccgaagaccccgaggtgcagatcagctggttcgtggatggaaagcagatgcagaccgccaagacccaaccccgggaagagcagttcaaaggcacctacagggtggtgagtgtgttgcccatcggccaccaggactggctgaaggggaagcaattcacatgcaaggttaataacaaggccctgcccagccccatcgagaggaccatcagcaaggccaggggccaggcccaccagccatctgtgtacgtgctgcccccatctagggaggaactgagcaagaacacagtcagccttacttgcctgatcaaggacttcttcccaccggacatagacgtggagtggcagagtaacggccagcaggagcccgagagcaagtataggaccacaccgccccaactggacgaggacggaagctacttcctctacagcaaattgagcgttgacaaaagcaggtggcagcgaggcgacaccttcatctgcgccgtgatgcacgaggctttgcataaccactacacccaggagagcctgtcccacagccccggatag

SEQ ID NO: 64 - protein, 290 aa, synthetic construct
  REGION 1..290: note = Fusion Protein
FVNQHLCGSDLVEALALVCGERGFFYTDPTGGGPRRGIVEQCCHSICSLYQLENYCNGGGGAGGGGDCPKCPAPEMLGGPSVFIFPPKPKDTLLIARTPEVTCVVVDLDPEDPEVQISWFVDGKQMQTAKTQPREEQFKGTYRVVSVLPIGHQDWLKGKQFTCKVNNKALPSPIERTISKARGQAHQPSVYVLPPSREELSKNTVSLTCLIKDFFPPDIDVEWQSNGQQEPESKYRTTPPQLDEDGSYFLYSKLSVDKSRWQRGDTFICAVMHEALHNHYTQESLSHSPG

SEQ ID NO: 65 - DNA, 930 bp, synthetic construct
  misc_feature 1..930: note = Fusion Protein DNA
  source 1..930: mol_type = other DNA
atggaatggagctgggtctttctcttcttcctgtcagtaacgactggtgtccactccttcgtgaaccagcacctgtgcggctcccacctggtggaagctctggctctcgtgtgcggcgagcggggcttcttctacaccgatcccactggaggcggtccacgcagaggcatcgtggaacagtgctgcacctccatctgctccctgtaccagctggaaaactactgcaatggcggaggtggtgcaggaggcggtggagactgccccaagtgccccgctcccgagatgctgggcggacccagcgtgttcatcttccctcccaagcccaaggacacactgctgatcgccaggaccccggaggtgacctgcgtggtggtggacctggatcccgaagaccccgaggtgcagatcagctggttcgtggatggaaagcagatgcagaccgccaagacccaaccccgggaagagcagttccaaggcacctacagggtggtgagtgtgttgcccatcggccaccaggactggctgaaggggaagcaattcacatgcaaggttaataacaaggccctgcccagccccatcgagaggaccatcagcaaggccaggggccaggcccaccagccatctgtgtacgtgctgcccccatctagggaggaactgagcaagaacacagtcagccttacttgcctgatcaaggacttcttcccaccggacatagacgtggagtggcagagtaacggccagcaggagcccgagagcaagtataggaccacaccgccccaactggacgaggacggaagctacttcctctacagcaaattgagcgttgacaaaagcaggtggcagcgaggcgacaccttcatctgcgccgtgatgcacgaggctttgcataaccactacacccaggagagcctgtcccacagccccggatag

SEQ ID NO: 66 - protein, 290 aa, synthetic construct
  REGION 1..290: note = Fusion Protein
FVNQHLCGSHLVEALALVCGERGFFYTDPTGGGPRRGIVEQCCTSICSLYQLENYCNGGGGAGGGGDCPKCPAPEMLGGPSVFIFPPKPKDTLLIARTPEVTCVVVDLDPEDPEVQISWFVDGKQMQTAKTQPREEQFQGTYRVVSVLPIGHQDWLKGKQFTCKVNNKALPSPIERTISKARGQAHQPSVYVLPPSREELSKNTVSLTCLIKDFFPPDIDVEWQSNGQQEPESKYRTTPPQLDEDGSYFLYSKLSVDKSRWQRGDTFICAVMHEALHNHYTQESLSHSPG

SEQ ID NO: 67 - DNA, 927 bp, synthetic construct
  misc_feature 1..927: note = Fusion Protein DNA
  source 1..927: mol_type = other DNA
atggaatggagctgggtctttctcttcttcctgtcagtaacgactggtgtccactccttcgtgaaccagcacctgtgcggctcccacctggtgcaagctctgtatctcgtgtgcggcgagcggggcttcttctacaccgatcccactggaggcggtccacgcagaggcatcgtggaacagtgctgcacctccatctgctccctgtaccagctggaaaactactgcggcggaggtggtgcaggaggcggtggagactgccccaagtgccccgctcccgagatgctgggcggacccagcgtgttcatcttccctcccaagcccaaggacacactgctgatcgccaggaccccggaggtgacctgcgtggtggtggacctggatcccgaagaccccgaggtgcagatcagctggttcgtggatggaaagcagatgcagaccgccaagacccaaccccgggaagagcagttcagcggcacctacagggtggtgagtgtgttgcccatcggccaccaggactggctgaaggggaagcaattcacatgcaaggttaataacaaggccctgcccagccccatcgagaggaccatcagcaaggccaggggccaggcccaccagccatctgtgtacgtgctgcccccatctagggaggaactgagcaagaacacagtcagccttacttgcctgatcaaggacttcttcccaccggacatagacgtggagtggcagagtaacggccagcaggagcccgagagcaagtataggaccacaccgccccaactggacgaggacggaagctacttcctctacagcaaattgagcgttgacaaaagcaggtggcagcgaggcgacaccttcatctgcgccgtgatgcacgaggctttgcataaccactacacccaggagagcctgtcccacagccccggatag

SEQ ID NO: 68 - protein, 289 aa, synthetic construct
  REGION 1..289: note = Fusion Protein
FVNQHLCGSHLVQALYLVCGERGFFYTDPTGGGPRRGIVEQCCTSICSLYQLENYCGGGGAGGGGDCPKCPAPEMLGGPSVFIFPPKPKDTLLIARTPEVTCVVVDLDPEDPEVQISWFVDGKQMQTAKTQPREEQFSGTYRVVSVLPIGHQDWLKGKQFTCKVNNKALPSPIERTISKARGQAHQPSVYVLPPSREELSKNTVSLTCLIKDFFPPDIDVEWQSNGQQEPESKYRTTPPQLDEDGSYFLYSKLSVDKSRWQRGDTFICAVMHEALHNHYTQESLSHSPG

SEQ ID NO: 69 - DNA, 927 bp, synthetic construct
  misc_feature 1..927: note = Fusion Protein DNA
  source 1..927: mol_type = other DNA
atggaatggagctgggtctttctcttcttcctgtcagtaacgactggtgtccactccttcgtgaaccagcacctgtgcggctccgagctggtggaagctctggctctcgtgtgcggcgagcggggcttcttctacaccgatcccactggaggcggtccacgcagaggcatcgtggaacagtgctgcacatccatctgctccctgtaccagctggaaaactactgcggcggaggtggtgcaggaggcggtggagactgccccaagtgccccgctcccgagatgctgggcggacccagcgtgttcatcttccctcccaagcccaaggacacactgctgatcgccaggaccccggaggtgacctgcgtggtggtggacctggatcccgaagaccccgaggtgcagatcagctggttcgtggatggaaagcagatgcagaccgccaagacccaaccccgggaagagcagttcagcggcacctacagggtggtgagtgtgttgcccatcggccaccaggactggctgaaggggaagcaattcacatgcaaggttaataacaaggccctgcccagccccatcgagaggaccatcagcaaggccaggggccaggcccaccagccatctgtgtacgtgctgcccccatctagggaggaactgagcaagaacacagtcagccttacttgcctgatcaaggacttcttcccaccggacatagacgtggagtggcagagtaacggccagcaggagcccgagagcaagtataggaccacaccgccccaactggacgaggacggaagctacttcctctacagcaaattgagcgttgacaaaagcaggtggcagcgaggcgacaccttcatctgcgccgtgatgcacgaggctttgcataaccactacacccaggagagcctgtcccacagccccggatag

SEQ ID NO: 70 - protein, 289 aa, synthetic construct
  REGION 1..289: note = Fusion Protein
FVNQHLCGSELVEALALVCGERGFFYTDPTGGGPRRGIVEQCCTSICSLYQLENYCGGGGAGGGGDCPKCPAPEMLGGPSVFIFPPKPKDTLLIARTPEVTCVVVDLDPEDPEVQISWFVDGKQMQTAKTQPREEQFSGTYRVVSVLPIGHQDWLKGKQFTCKVNNKALPSPIERTISKARGQAHQPSVYVLPPSREELSKNTVSLTCLIKDFFPPDIDVEWQSNGQQEPESKYRTTPPQLDEDGSYFLYSKLSVDKSRWQRGDTFICAVMHEALHNHYTQESLSHSPG

SEQ ID NO: 71 - DNA, 927 bp, synthetic construct
  misc_feature 1..927: note = Fusion Protein DNA
  source 1..927: mol_type = other DNA
atggaatggagctgggtctttctcttcttcctgtcagtaacgactggtgtccactccttcgtgaaccagcacctgtgcggctcccacctggtggaagctctggctctcgtgtgcggcgaggccggcttcttctacaccgatcccactggaggcggtccacgcagaggcatcgtggaacagtgctgcacctccatctgctccctgtaccagctggaaaactactgcggcggaggtggtgcaggaggcggtggagactgccccaagtgccccgctcccgagatgctgggcggacccagcgtgttcatcttccctcccaagcccaaggacacactgctgatcgccaggaccccggaggtgacctgcgtggtggtggacctggatcccgaagaccccgaggtgcagatcagctggttcgtggatggaaagcagatgcagaccgccaagacccaaccccgggaagagcagttcagcggcacctacagggtggtgagtgtgttgcccatcggccaccaggactggctgaaggggaagcaattcacatgcaaggttaataacaaggccctgcccagccccatcgagaggaccatcagcaaggccaggggccaggcccaccagccatctgtgtacgtgctgcccccatctagggaggaactgagcaagaacacagtcagccttacttgcctgatcaaggacttcttcccaccggacatagacgtggagtggcagagtaacggccagcaggagcccgagagcaagtataggaccacaccgccccaactggacgaggacggaagctacttcctctacagcaaattgagcgttgacaaaagcaggtggcagcgaggcgacaccttcatctgcgccgtgatgcacgaggctttgcataaccactacacccaggagagcctgtcccacagccccggatag

SEQ ID NO: 72 - protein, 289 aa, synthetic construct
  REGION 1..289: note = Fusion Protein
FVNQHLCGSHLVEALALVCGEAGFFYTDPTGGGPRRGIVEQCCTSICSLYQLENYCGGGGAGGGGDCPKCPAPEMLGGPSVFIFPPKPKDTLLIARTPEVTCVVVDLDPEDPEVQISWFVDGKQMQTAKTQPREEQFSGTYRVVSVLPIGHQDWLKGKQFTCKVNNKALPSPIERTISKARGQAHQPSVYVLPPSREELSKNTVSLTCLIKDFFPPDIDVEWQSNGQQEPESKYRTTPPQLDEDGSYFLYSKLSVDKSRWQRGDTFICAVMHEALHNHYTQESLSHSPG

SEQ ID NO: 73 - DNA, 927 bp, synthetic construct
  misc_feature 1..927: note = Fusion Protein DNA
  source 1..927: mol_type = other DNA
atggaatggagctgggtctttctcttcttcctgtcagtaacgactggtgtccactccttcgtgaaccagcacctgtgcggctcccacctggtggaagctctggctctcgtgtgcggcgagcggggcttctactacaccgatcccactggaggcggtccacgcagaggcatcgtggaacagtgctgcacctccatctgctccctgtaccagctggaaaactactgcggcggaggtggtgcaggaggcggtggagactgccccaagtgccccgctcccgagatgctgggcggacccagcgtgttcatcttccctcccaagcccaaggacacactgctgatcgccaggaccccggaggtgacctgcgtggtggtggacctggatcccgaagaccccgaggtgcagatcagctggttcgtggatggaaagcagatgcagaccgccaagacccaaccccgggaagagcagttcagcggcacctacagggtggtgagtgtgttgcccatcggccaccaggactggctgaaggggaagcaattcacatgcaaggttaataacaaggccctgcccagccccatcgagaggaccatcagcaaggccaggggccaggcccaccagccatctgtgtacgtgctgcccccatctagggaggaactgagcaagaacacagtcagccttacttgcctgatcaaggacttcttcccaccggacatagacgtggagtggcagagtaacggccagcaggagcccgagagcaagtataggaccacaccgccccaactggacgaggacggaagctacttcctctacagcaaattgagcgttgacaaaagcaggtggcagcgaggcgacaccttcatctgcgccgtgatgcacgaggctttgcataaccactacacccaggagagcctgtcccacagccccggatag

SEQ ID NO: 74 - protein, 289 aa, synthetic construct
  REGION 1..289: note = Fusion Protein DNA
FVNQHLCGSHLVEALALVCGERGFYYTDPTGGGPRRGIVEQCCTSICSLYQLENYCGGGGAGGGGDCPKCPAPEMLGGPSVFIFPPKPKDTLLIARTPEVTCVVVDLDPEDPEVQISWFVDGKQMQTAKTQPREEQFSGTYRVVSVLPIGHQDWLKGKQFTCKVNNKALPSPIERTISKARGQAHQPSVYVLPPSREELSKNTVSLTCLIKDFFPPDIDVEWQSNGQQEPESKYRTTPPQLDEDGSYFLYSKLSVDKSRWQRGDTFICAVMHEALHNHYTQESLSHSPG

SEQ ID NO: 75 - DNA, 927 bp, synthetic construct
  misc_feature 1..927: note = Fusion Protein DNA
  source 1..927: mol_type = other DNA
atggaatggagctgggtctttctcttcttcctgtcagtaacgactggtgtccactccttcgtgaaccagcacctgtgcggctcccacctggtggaagctctggctctcgtgtgcggcgagcggggcttcttctacaccgatcccactggaggcggtccacgcagaggcatcgtggaacagtgctgcacctccatctgctccctgtaccagctggaaaactactgcggcggaggtggtgcaggaggcggtggagactgccccaagtgccccgctcccgagatgctgggcggacccagcgtgttcatcttccctcccaagcccaaggacacactgctgatcgccaggaccccggaggtgacctgcgtggtggtggacctggatcccgaagaccccgaggtgcagatcagctggttcgtggatggaaagcagatgcagaccgccaagacccaaccccgggaagagcagttcagcggcacctacagggtggtgagtgtgttgcccatcggccaccaggactggctgaaggggaagcaattcacatgcaaggttaataacaaggccctgcccagccccatcgagaggaccatcagcaaggccaggggccaggcccaccagccatctgtgtacgtgctgcccccatctagggaggaactgagcaagaacacagtcagccttacttgcctgatcaaggacttcttcccaccggacatagacgtggagtggcagagtaacggccagcaggagcccgagagcaagtataggaccacaccgccccaactggacgaggacggaagctacttcctctacagcaaattgagcgttgacaaaagcaggtggcagcgaggcgacaccttcatctgcgccgtgatgcacgaggctttgcataaccactacacccaggagagcctgtcccacagccccggatag

SEQ ID NO: 76 - protein, 289 aa, synthetic construct
  REGION 1..289: note = Fusion Protein
FVNQHLCGSHLVEALALVCGERGFFYTDPTGGGPRRGIVEQCCTSICSLYQLENYCGGGGAGGGGDCPKCPAPEMLGGPSVFIFPPKPKDTLLIARTPEVTCVVVDLDPEDPEVQISWFVDGKQMQTAKTQPREEQFSGTYRVVSVLPIGHQDWLKGKQFTCKVNNKALPSPIERTISKARGQAHQPSVYVLPPSREELSKNTVSLTCLIKDFFPPDIDVEWQSNGQQEPESKYRTTPPQLDEDGSYFLYSKLSVDKSRWQRGDTFICAVMHEALHNHYTQESLSHSPG

SEQ ID NO: 77 - DNA, 936 bp, synthetic construct
  misc_feature 1..936: note = Fusion Protein DNA
  source 1..936: mol_type = other DNA
atggaatggagctgggtctttctcttcttcctgtcagtaacgactggtgtccactccttcgtgaaccagcacctgtgcggctcccacctggtgcaagctctgtatctcgtgtgcggcgagcggggcttcttctacaccgatcccactcagaggggcggtggcggagggcaaagaggcatcgtggaacagtgctgcacatccatctgctccctgtaccagctggaaaactactgcggcggaggtggtgcaggaggcggtggagactgccccaagtgccccgctcccgagatgctgggcggacccagcgtgttcatcttccctcccaagcccaaggacacactgctgatcgccaggaccccggaggtgacctgcgtggtggtggacctggatcccgaagaccccgaggtgcagatcagctggttcgtggatggaaagcagatgcagaccgccaagacccaaccccgggaagagcagttcagcggcacctacagggtggtgagtgtgttgcccatcggccaccaggactggctgaaggggaagcaattcacatgcaaggttaataacaaggccctgcccagccccatcgagaggaccatcagcaaggccaggggccaggcccaccagccatctgtgtacgtgctgcccccatctagggaggaactgagcaagaacacagtcagccttacttgcctgatcaaggacttcttcccaccggacatagacgtggagtggcagagtaacggccagcaggagcccgagagcaagtataggaccacaccgccccaactggacgaggacggaagctacttcctctacagcaaattgagcgttgacaaaagcaggtggcagcgaggcgacaccttcatctgcgccgtgatgcacgaggctttgcataaccactacacccaggagagcctgtcccacagccccggatag

SEQ ID NO: 78 - protein, 292 aa, synthetic construct
  REGION 1..292: note = Fusion Protein
FVNQHLCGSHLVQALYLVCGERGFFYTDPTQRGGGGGQRGIVEQCCTSICSLYQLENYCGGGGAGGGGDCPKCPAPEMLGGPSVFIFPPKPKDTLLIARTPEVTCVVVDLDPEDPEVQISWFVDGKQMQTAKTQPREEQFSGTYRVVSVLPIGHQDWLKGKQFTCKVNNKALPSPIERTISKARGQAHQPSVYVLPPSREELSKNTVSLTCLIKDFFPPDIDVEWQSNGQQEPESKYRTTPPQLDEDGSYFLYSKLSVDKSRWQRGDTFICAVMHEALHNHYTQESLSHSPG

SEQ ID NO: 79 - DNA, 942 bp, synthetic construct
  misc_feature 1..942: note = Fusion Protein DNA
  source 1..942: mol_type = other DNA
atggaatggagctgggtctttctcttcttcctgtcagtaacgactggtgtccactccttcgtgaaccagcacctgtgcggctcccacctggtggaagctctggctctcgtgtgcggcgagcggggcttcttctacaccgatcccactgggggtggcggaggaggttctggtggcggcggaggcatcgtggaacagtgctgcacctccatctgctccctgtaccagctggaaaactactgcggcggaggtggtgcaggaggcggtggagactgccccaagtgccccgctcccgagatgctgggcggacccagcgtgttcatcttccctcccaagcccaaggacacactgctgatcgccaggaccccggaggtgacctgcgtggtggtggacctggatcccgaagaccccgaggtgcagatcagctggttcgtggatggaaagcagatgcagaccgccaagacccaaccccgggaagagcagttcagcggcacctacagggtggtgagtgtgttgcccatcggccaccaggactggctgaaggggaagcaattcacatgcaaggttaataacaaggccctgcccagccccatcgagaggaccatcagcaaggccaggggccaggcccaccagccatctgtgtacgtgctgcccccatctagggaggaactgagcaagaacacagtcagccttacttgcctgatcaaggacttcttcccaccggacatagacgtggagtggcagagtaacggccagcaggagcccgagagcaagtataggaccacaccgccccaactggacgaggacggaagctacttcctctacagcaaattgagcgttgacaaaagcaggtggcagcgaggcgacaccttcatctgcgccgtgatgcacgaggctttgcataaccactacacccaggagagcctgtcccacagccccggatag

SEQ ID NO: 80 - protein, 294 aa, synthetic construct
  REGION 1..294: note = Fusion Protein
FVNQHLCGSHLVEALALVCGERGFFYTDPTGGGGGGSGGGGGIVEQCCTSICSLYQLENYCGGGGAGGGGDCPKCPAPEMLGGPSVFIFPPKPKDTLLIARTPEVTCVVVDLDPEDPEVQISWFVDGKQMQTAKTQPREEQFSGTYRVVSVLPIGHQDWLKGKQFTCKVNNKALPSPIERTISKARGQAHQPSVYVLPPSREELSKNTVSLTCLIKDFFPPDIDVEWQSNGQQEPESKYRTTPPQLDEDGSYFLYSKLSVDKSRWQRGDTFICAVMHEALHNHYTQESLSHSPG

SEQ ID NO: 81 - DNA, 930 bp, synthetic construct
  misc_feature 1..930: note = Fusion Protein DNA
  source 1..930: mol_type = other DNA
atggaatggagctgggtctttctcttcttcctgtcagtaacgactggtgtccactccttcgtgaaccagcacctctgcggcagccacctggtggaggccttggccctggtgtgcggcgagaggggcttcttctacaccgatccaggtggcggtgggggaggtggcggagggatcgtggagcagtgctgcaccagcatctgcagcctgtaccaactggaaaactactgcggcggaggtggtgcaggaggcggtggagactgccccaagtgccccgctcccgagatgctgggcggacccagcgtgttcatcttccctcccaagcccaaggacacactgctgatcgccaggaccccggaggtgacctgcgtggtggtggacctggatcccgaagaccccgaggtgcagatcagctggttcgtggatggaaagcagatgcagaccgccaagacccaaccccgggaagagcagttcagcggcacctacagggtggtgagtgtgttgcccatcggccaccaggactggctgaaggggaagcaattcacatgcaaggttaataacaaggccctgcccagccccatcgagaggaccatcagcaaggccaggggccaggcccaccagccatctgtgtacgtgctgcccccatctagggaggaactgagcaagaacacagtcagccttacttgcctgatcaaggacttcttcccaccggacatagacgtggagtggcagagtaacggccagcaggagcccgagagcaagtataggaccacaccgccccaactggacgaggacggaagctacttcctctacagcaaattgagcgttgacaaaagcaggtggcagcgaggcgacaccttcatctgcgccgtgatgcacgaggctttgcataaccactacacccaggagagcctgtcccacagccccggatag

SEQ ID NO: 82 - protein, 290 aa, synthetic construct
  REGION 1..290: note = Fusion Protein
FVNQHLCGSHLVEALALVCGERGFFYTDPGGGGGGGGGIVEQCCTSICSLYQLENYCGGGGAGGGGDCPKCPAPEMLGGPSVFIFPPKPKDTLLIARTPEVTCVVVDLDPEDPEVQISWFVDGKQMQTAKTQPREEQFSGTYRVVSVLPIGHQDWLKGKQFTCKVNNKALPSPIERTISKARGQAHQPSVYVLPPSREELSKNTVSLTCLIKDFFPPDIDVEWQSNGQQEPESKYRTTPPQLDEDGSYFLYSKLSVDKSRWQRGDTFICAVMHEALHNHYTQESLSHSPG

SEQ ID NO: 83 - DNA, 927 bp, synthetic construct
  misc_feature 1..927: note = Fusion Protein DNA
  source 1..927: mol_type = other DNA
atggaatggagctgggtctttctcttcttcctgtcagtaacgactggtgtccactccttcgtgaaccagcacctctgcggcagccacctggtggaggccttggccctggtgtgcggcgagaggggcttcttctacaccccaggtggcggtgggggaggtggcggagggatcgtggagcagtgctgcaccagcatctgcagcctgtaccaactggaaaactactgcggcggaggtggtgcaggaggcggtggagactgccccaagtgccccgctcccgagatgctgggcggacccagcgtgttcatcttccctcccaagcccaaggacacactgctgatcgccaggaccccggaggtgacctgcgtggtggtggacctggatcccgaagaccccgaggtgcagatcagctggttcgtggatggaaagcagatgcagaccgccaagacccaaccccgggaagagcagttcagcggcacctacagggtggtgagtgtgttgcccatcggccaccaggactggctgaaggggaagcaattcacatgcaaggttaataacaaggccctgcccagccccatcgagaggaccatcagcaaggccaggggccaggcccaccagccatctgtgtacgtgctgcccccatctagggaggaactgagcaagaacacagtcagccttacttgcctgatcaaggacttcttcccaccggacatagacgtggagtggcagagtaacggccagcaggagcccgagagcaagtataggaccacaccgccccaactggacgaggacggaagctacttcctctacagcaaattgagcgttgacaaaagcaggtggcagcgaggcgacaccttcatctgcgccgtgatgcacgaggctttgcataaccactacacccaggagagcctgtcccacagccccggatag

SEQ ID NO: 84 - protein, 289 aa, synthetic construct
  REGION 1..289: note = Fusion Protein
FVNQHLCGSHLVEALALVCGERGFFYTPGGGGGGGGGIVEQCCTSICSLYQLENYCGGGGAGGGGDCPKCPAPEMLGGPSVFIFPPKPKDTLLIARTPEVTCVVVDLDPEDPEVQISWFVDGKQMQTAKTQPREEQFSGTYRVVSVLPIGHQDWLKGKQFTCKVNNKALPSPIERTISKARGQAHQPSVYVLPPSREELSKNTVSLTCLIKDFFPPDIDVEWQSNGQQEPESKYRTTPPQLDEDGSYFLYSKLSVDKSRWQRGDTFICAVMHEALHNHYTQESLSHSPG

SEQ ID NO: 85 - DNA, 963 bp, synthetic construct
  misc_feature 1..963: note = Fusion Protein DNA
  source 1..963: mol_type = other DNA
atggaatggagctgggtctttctcttcttcctgtcagtaacgactggtgtccactccttcgtgaaccagcacctgtgcggctcccacctggtggaagctctggctctcgtgtgcggcgagcggggcttcttctacaccgatcccactggaggcggtccacgcagaggcatcgtggaacagtgctgcacctccatctgctccctgtaccagctggaaaactactgcggtggcggaggtggtcaaggaggcggtggacagggtggaggtgggcagggaggaggcgggggagactgccccaagtgccccgctcccgagatgctgggcggacccagcgtgttcatcttccctcccaagcccaaggacacactgctgatcgccaggaccccggaggtgacctgcgtggtggtggacctggatcccgaagaccccgaggtgcagatcagctggttcgtggatggaaagcagatgcagaccgccaagacccaaccccgggaagagcagttcagcggcacctacagggtggtgagtgtgttgcccatcggccaccaggactggctgaaggggaagcaattcacatgcaaggttaataacaaggccctgcccagccccatcgagaggaccatcagcaaggccaggggccaggcccaccagccatctgtgtacgtgctgcccccatctagggaggaactgagcaagaacacagtcagccttacttgcctgatcaaggacttcttcccaccggacatagacgtggagtggcagagtaacggccagcaggagcccgagagcaagtataggaccacaccgccccaactggacgaggacggaagctacttcctctacagcaaattgagcgttgacaaaagcaggtggcagcgaggcgacaccttcatctgcgccgtgatgcacgaggctttgcataaccactacacccaggagagcctgtcccacagccccggatag

SEQ ID NO: 86 - protein, 301 aa, synthetic construct
  REGION 1..301: note = Fusion Protein
FVNQHLCGSHLVEALALVCGERGFFYTDPTGGGPRRGIVEQCCTSICSLYQLENYCGGGGGQGGGGQGGGGQGGGGGDCPKCPAPEMLGGPSVFIFPPKPKDTLLIARTPEVTCVVVDLDPEDPEVQISWFVDGKQMQTAKTQPREEQFSGTYRVVSVLPIGHQDWLKGKQFTCKVNNKALPSPIERTISKARGQAHQPSVYVLPPSREELSKNTVSLTCLIKDFFPPDIDVEWQSNGQQEPESKYRTTPPQLDEDGSYFLYSKLSVDKSRWQRGDTFICAVMHEALHNHYTQESLSHSPG

SEQ ID NO: 87 - DNA, 927 bp, synthetic construct
  misc_feature 1..927: note = Fusion Protein DNA
  source 1..927: mol_type = other DNA
atggaatggagctgggtctttctcttcttcctgtcagtaacgactggtgtccactccttcgtgaaccagcacctctgcggcagccacctggtggaggccttggccctggtgtgcggcgagaggggcttcttctacacccagggtggcggtgggggaggtggcggagggatcgtggagcagtgctgcaccagcatctgcagcctgtaccaactggaaaactactgcggcggaggtggtgcaggaggcggtggagactgccccaagtgccccgctcccgagatgctgggcggacccagcgtgttcatcttccctcccaagcccaaggacacactgctgatcgccaggaccccggaggtgacctgcgtggtggtggacctggatcccgaagaccccgaggtgcagatcagctggttcgtggatggaaagcagatgcagaccgccaagacccaaccccgggaagagcagttcagcggcacctacagggtggtgagtgtgttgcccatcggccaccaggactggctgaaggggaagcaattcacatgcaaggttaataacaaggccctgcccagccccatcgagaggaccatcagcaaggccaggggccaggcccaccagccatctgtgtacgtgctgcccccatctagggaggaactgagcaagaacacagtcagccttacttgcctgatcaaggacttcttcccaccggacatagacgtggagtggcagagtaacggccagcaggagcccgagagcaagtataggaccacaccgccccaactggacgaggacggaagctacttcctctacagcaaattgagcgttgacaaaagcaggtggcagcgaggcgacaccttcatctgcgccgtgatgcacgaggctttgcataaccactacacccaggagagcctgtcccacagccccggatag

SEQ ID NO: 88 - protein, 289 aa, synthetic construct
  REGION 1..289: note = Fusion Protein
FVNQHLCGSHLVEALALVCGERGFFYTQGGGGGGGGGIVEQCCTSICSLYQLENYCGGGGAGGGGDCPKCPAPEMLGGPSVFIFPPKPKDTLLIARTPEVTCVVVDLDPEDPEVQISWFVDGKQMQTAKTQPREEQFSGTYRVVSVLPIGHQDWLKGKQFTCKVNNKALPSPIERTISKARGQAHQPSVYVLPPSREELSKNTVSLTCLIKDFFPPDIDVEWQSNGQQEPESKYRTTPPQLDEDGSYFLYSKLSVDKSRWQRGDTFICAVMHEALHNHYTQESLSHSPG

SEQ ID NO: 89 - DNA, 966 bp, synthetic construct
  misc_feature 1..966: note = Fusion Protein DNA
  source 1..966: mol_type = other DNA
atggaatggagctgggtctttctcttcttcctgtcagtaacgactggtgtccactccttcgtgaaccagcacctgtgcggctcccacctggtggaagctctggaactcgtgtgcggcgagcggggcttcttctacacccctaagacaggaggttctggtggcggcggaggcatcgtggaacagtgctgcacctccacctgctccctggaccagctggaaaactactgcggtggcggaggtggtcaaggaggcggtggacagggtggaggtgggcagggaggaggcgggggagactgccccaagtgccccgctcccgagatgctgggcggacccagcgtgttcatcttccctcccaagcccaaggacacactgctgatcgccaggaccccggaggtgacctgcgtggtggtggacctggatcccgaagaccccgaggtgcagatcagctggttcgtggatggaaagcagatgcagaccgccaagacccaaccccgggaagagcagttcaacggcacctacagggtggtgagtgtgttgcccatcggccaccaggactggctgaaggggaagcaattcacatgcaaggttaataacaaggccctgcccagccccatcgagaggaccatcagcaaggccaggggccaggcccaccagccatctgtgtacgtgctgcccccatctagggaggaactgagcaagaacacagtcagccttacttgcctgatcaaggacttcttcccaccggacatagacgtggagtggcagagtaacggccagcaggagcccgagagcaagtataggaccacaccgccccaactggacgaggacggaagctacttcctctacagcaaattgagcgttgacaaaagcaggtggcagcgaggcgacaccttcatctgcgccgtgatgcacgaggctttgcataaccactacacccaggagagcctgtcccacagccccggatag

SEQ ID NO: 90 - protein, 302 aa, synthetic construct
  REGION 1..302: note = Fusion Protein
FVNQHLCGSHLVEALELVCGERGFFYTPKTGGSGGGGGIVEQCCTSTCSLDQLENYCGGGGGQGGGGQGGGGQGGGGGDCPKCPAPEMLGGPSVFIFPPKPKDTLLIARTPEVTCVVVDLDPEDPEVQISWFVDGKQMQTAKTQPREEQFNGTYRVVSVLPIGHQDWLKGKQFTCKVNNKALPSPIERTISKARGQAHQPSVYVLPPSREELSKNTVSLTCLIKDFFPPDIDVEWQSNGQQEPESKYRTTPPQLDEDGSYFLYSKLSVDKSRWQRGDTFICAVMHEALHNHYTQESLSHSPG

SEQ ID NO: 91 - DNA, 969 bp, synthetic construct
  misc_feature 1..969: note = Fusion Protein DNA
  source 1..969: mol_type = other DNA
atggaatggagctgggtctttctcttcttcctgtcagtaacgactggtgtccactccttcgtgaaccagcacctgtgcggctcccacctggtggaagctctggaactcgtgtgcggcgagcggggcttccactacgggggtggcggaggaggttctggtggcggcggaggcatcgtggaacagtgctgcacctccacctgctccctggaccagctggaaaactactgcaaccatggcggaggtggtcaaggaggcggtggacagggtggaggtgggcagggaggaggcgggggagactgccccaagtgccccgctcccgagatgctgggcggacccagcgtgttcatcttccctcccaagcccaaggacacactgctgatcgccaggaccccggaggtgacctgcgtggtggtggacctggatcccgaagaccccgaggtgcagatcagctggttcgtggatggaaagcagatgcagaccgccaagacccaaccccgggaagagcagttcaacggcacctacagggtggtgagtgtgttgcccatcggccaccaggactggctgaaggggaagcaattcacatgcaaggttaataacaaggccctgcccagccccatcgagaggaccatcagcaaggccaggggccaggcccaccagccatctgtgtacgtgctgcccccatctagggaggaactgagcaagaacacagtcagccttacttgcctgatcaaggacttcttcccaccggacatagacgtggagtggcagagtaacggccagcaggagcccgagagcaagtataggaccacaccgccccaactggacgaggacggaagctacttcctctacagcaaattgagcgttgacaaaagcaggtggcagcgaggcgacaccttcatctgcgccgtgatgcacgaggctttgcataaccactacacccaggagagcctgtcccacagccccggatag

SEQ ID NO: 92 - protein, 303 aa, synthetic construct
  REGION 1..303: note = Fusion Protein
FVNQHLCGSHLVEALELVCGERGFHYGGGGGGSGGGGGIVEQCCTSTCSLDQLENYCNHGGGGQGGGGQGGGGQGGGGGDCPKCPAPEMLGGPSVFIFPPKPKDTLLIARTPEVTCVVVDLDPEDPEVQISWFVDGKQMQTAKTQPREEQFNGTYRVVSVLPIGHQDWLKGKQFTCKVNNKALPSPIERTISKARGQAHQPSVYVLPPSREELSKNTVSLTCLIKDFFPPDIDVEWQSNGQQEPESKYRTTPPQLDEDGSYFLYSKLSVDKSRWQRGDTFICAVMHEALHNHYTQESLSHSPG

SEQ ID NO: 93 - DNA, 966 bp, synthetic construct
  misc_feature 1..966: note = Fusion Protein DNA
  source 1..966: mol_type = other DNA
atggaatggagctgggtctttctcttcttcctgtcagtaacgactggtgtccactccttcgtgaaccagcacctgtgcggctcccacctggtggaagctctggaactcgtgtgcggcgagcggggcttcttctacgggggtggcggaggaggttctggtggcggcggaggcatcgtggaacagtgctgcacctccacctgctccctggaccagctggaaaactactgcggtggcggaggtggtcaaggaggcggtggacagggtggaggtgggcagggaggaggcgggggagactgccccaagtgccccgctcccgagatgctgggcggacccagcgtgttcatcttccctcccaagcccaaggacacactgctgatcgccaggaccccggaggtgacctgcgtggtggtggacctggatcccgaagaccccgaggtgcagatcagctggttcgtggatggaaagcagatgcagaccgccaagacccaaccccgggaagagcagttcaacggcacctacagggtggtgagtgtgttgcccatcggccaccaggactggctgaaggggaagcaattcacatgcaaggttaataacaaggccctgcccagccccatcgagaggaccatcagcaaggccaggggccaggcccaccagccatctgtgtacgtgctgcccccatctagggaggaactgagcaagaacacagtcagccttacttgcctgatcaaggacttcttcccaccggacatagacgtggagtggcagagtaacggccagcaggagcccgagagcaagtataggaccacaccgccccaactggacgaggacggaagctacttcctctacagcaaattgagcgttgacaaaagcaggtggcagcgaggcgacaccttcatctgcgccgtgatgcacgaggctttgcataaccactacacccaggagagcctgtcccacagccccggatag

SEQ ID NO: 94 - protein, 302 aa, synthetic construct
  REGION 1..302: note = Fusion Protein
FVNQHLCGSHLVEALELVCGERGFFYGGGGGGSGGGGGIVEQCCTSTCSLDQLENYCGGGGGQGGGGQGGGGQGGGGGDCPKCPAPEMLGGPSVFIFPPKPKDTLLIARTPEVTCVVVDLDPEDPEVQISWFVDGKQMQTAKTQPREEQFNGTYRVVSVLPIGHQDWLKGKQFTCKVNNKALPSPIERTISKARGQAHQPSVYVLPPSREELSKNTVSLTCLIKDFFPPDIDVEWQSNGQQEPESKYRTTPPQLDEDGSYFLYSKLSVDKSRWQRGDTFICAVMHEALHNHYTQESLSHSPG

SEQ ID NO: 95 - DNA, 978 bp, synthetic construct
  misc_feature 1..978: note = Fusion Protein DNA
  source 1..978: mol_type = other DNA
atggaatggagctgggtctttctcttcttcctgtcagtaacgactggtgtccactccttcgtgaaccagcacctgtgcggctcccacctggtggaagctctggaactcgtgtgcggcgagcggggcttccactacgggggtggcggaggaggttctggtggcggcggaggcatcgtggaacagtgctgcacctccacctgctccctggaccagctggaaaactactgcggtggcggaggtggtcaaggaggcggtggacagggtggaggtgggcagggaggaggcgggggacgctgcactgacacccctccatgccctgtgcccgagcccctgggtggccccagcgtactgatcttcccaccgaaacccaaggacatcctgaggatcacccgcaccccggaggtgacctgcgtggtgctggacctgggcagggaggaccccgaagtgcaaatcagctggttcgtggacggaaaggaggtgcacaccgccaagacccaatcaagggagcagcagttcaacggcacctacagggtggtgagcgtgttgcccatagagcaccaggactggctgaccggcaaggagttcaagtgccgcgtgaaccacattgatctccccagccccatcgagaggactatctccaaggcccgagggagggcccacaagcccagtgtatacgtgctgccgccctctccgaaggaactgagctctagcgacaccgtgagcatcacctgcctgatcaaggacttctaccctcccgacatagacgtagagtggcagagcaacggccagcaggagcccgaaaggaagcacaggatgaccccaccccaactggacgaggacggctcatactttctttatagcaagctgagtgtggacaagagcaggtggcagcagggcgaccctttcacttgcgccgtaatgcacgagaccctgcagaatcactacaccgacctgtcactgagccatagccccggatag

SEQ ID NO: 96 - protein, 306 aa, synthetic construct
  REGION 1..306: note = Fusion Protein
FVNQHLCGSHLVEALELVCGERGFHYGGGGGGSGGGGGIVEQCCTSTCSLDQLENYCGGGGGQGGGGQGGGGQGGGGGRCTDTPPCPVPEPLGGPSVLIFPPKPKDILRITRTPEVTCVVLDLGREDPEVQISWFVDGKEVHTAKTQSREQQFNGTYRVVSVLPIEHQDWLTGKEFKCRVNHIDLPSPIERTISKARGRAHKPSVYVLPPSPKELSSSDTVSITCLIKDFYPPDIDVEWQSNGQQEPERKHRMTPPQLDEDGSYFLYSKLSVDKSRWQQGDPFTCAVMHETLQNHYTDLSLSHSPG

SEQ ID NO: 97 - DNA, 969 bp, synthetic construct
  misc_feature 1..969: note = Fusion Protein DNA
  source 1..969: mol_type = other DNA
atggaatggagctgggtctttctcttcttcctgtcagtaacgactggtgtccactccttcgtgaaccagcacctgtgcggctcccacctggtggaagctctggaactcgtgtgcggcgagcggggcttccactacgggggtggcggaggaggttctggtggcggcggaggcatcgtggaacagtgctgcacctccacctgctccctggaccagctggaaaactactgcggtggcggaggtggtcaaggaggcggtggacagggtggaggtgggcagggaggaggcgggggatgcaacaactgcccgtgtccgggatgcggcctcctgggcggaccgagcgtgttcattttccctcctaagcccaaggacattctggtgaccgccaggacccccacggtgacctgcgtggtagtagatctcgatcccgaaaacccagaggtgcaaatcagctggttcgtggactctaagcaagtgcaaaccgccaacacgcaaccccgcgaggaacagagcaacggcacctacagggtggtgagcgtgctgcccatcgggcatcaggactggctgagcggcaagcagtttaaatgcaaggttaacaacaaggcactgcccagccccatcgaggagatcatcagcaagaccccgggacaggcccaccagcccaacgtgtacgtccttcctccgagccgcgacgagatgagcaagaacaccgtgacgctgacctgtttggtgaaggacttcttcccacccgagatcgacgtggagtggcaaagcaatggccagcaggagcccgagagcaaatacaggatgaccccaccccaactggatgaggatggcagctatttcctctacagcaaattgtccgtggacaaaagcaggtggcagaggggcgacaccttcatctgcgccgtcatgcacgaggcccttcacaatcactacacccagatcagcctgagccactctcccggatag

SEQ ID NO: 98 - protein, 303 aa, synthetic construct
  REGION 1..303: note = Fusion Protein
FVNQHLCGSHLVEALELVCGERGFHYGGGGGGSGGGGGIVEQCCTSTCSLDQLENYCGGGGGQGGGGQGGGGQGGGGGCNNCPCPGCGLLGGPSVFIFPPKPKDILVTARTPTVTCVVVDLDPENPEVQISWFVDSKQVQTANTQPREEQSNGTYRVVSVLPIGHQDWLSGKQFKCKVNNKALPSPIEEIISKTPGQAHQPNVYVLPPSRDEMSKNTVTLTCLVKDFFPPEIDVEWQSNGQQEPESKYRMTPPQLDEDGSYFLYSKLSVDKSRWQRGDTFICAVMHEALHNHYTQISLSHSPG

SEQ ID NO: 99 - DNA, 969 bp, synthetic construct
  misc_feature 1..969: note = Fusion Protein DNA
  source 1..969: mol_type = other DNA
atggaatggagctgggtctttctcttcttcctgtcagtaacgactggtgtccactccttcgtgaaccagcacctgtgcggctcccacctggtggaagctctggaactcgtgtgcggcgagcggggcttccactacgggggtggcggaggaggttctggtggcggcggaggcatcgtggaacagtgctgcacctccacctgctccctggaccagctggaaaactactgcggtggcggaggtggtcaaggaggcggtggacagggtggaggtgggcagggaggaggcgggggatgcatcagcccctgccccgtgccggagagcctgggtggccctagcgtgttcatattccctcccaagcccaaggacatcctgaggatcaccaggacccccgagatcacctgtgtggtgctggatcttggcagggaagaccccgaagtccagatcagctggttcgtggatggcaaggaggtgcacaccgccaagacccagccgagggagcagcagttcaactccacctacagggtggtgagcgtgctgcctatcgagcatcaggactggctgaccggcaaagagttcaagtgcagggtgaaccacatcggcctgcccagccccatcgagaggaccatcagcaaagccaggggccaggcccaccagcccagtgtgtacgtgcttccccctagcccaaaggaactgagtagcagcgataccgtgaccctgacctgcctgatcaaggactttttcccgccagaaatagacgtggagtggcagagcaacggccagccggagcccgagagcaaataccacaccaccgcccctcaactggacgaggacgggagctacttcctgtatagcaagctgagcgttgacaagagcaggtggcaacagggcgacaccttcacctgcgccgtgatgcacgaagctctgcaaaaccactacaccgacctgtcactgagccatagccccggatag

SEQ ID NO: 100 - protein, 303 aa, synthetic construct
  REGION 1..303: note = Fusion Protein
FVNQHLCGSHLVEALELVCGERGFHYGGGGGGSGGGGGIVEQCCTSTCSLDQLENYCGGGGGQGGGGQGGGGQGGGGGCISPCPVPESLGGPSVFIFPPKPKDILRITRTPEITCVVLDLGREDPEVQISWFVDGKEVHTAKTQPREQQFNSTYRVVSVLPIEHQDWLTGKEFKCRVNHIGLPSPIERTISKARGQAHQPSVYVLPPSPKELSSSDTVTLTCLIKDFFPPEIDVEWQSNGQPEPESKYHTTAPQLDEDGSYFLYSKLSVDKSRWQQGDTFTCAVMHEALQNHYTDLSLSHSPG

SEQ ID NO: 101 - DNA, 966 bp, synthetic construct
  misc_feature 1..966: note = Fusion Protein DNA
  source 1..966: mol_type = other DNA
atggaatggagctgggtctttctcttcttcctgtcagtaacgactggtgtccactccttcgtgaaccagcacctgtgcggctcccacctggtggaagctctggaactcgtgtgcggcgagcggggcttccactacgggggtggcggaggaggttctggtggcggcggaggcatcgtggaacagtgctgcacctccacctgctccctggaccagctggaaaactactgcggtggcggaggtggtcaaggaggcggtggacagggtggaggtgggcagggaggaggcgggggagactgccccaagtgccccgctcccgagatgctgggcggacccagcgtgttcatcttccctcccaagcccaaggacacactgctgatcgccaggaccccggaggtgacctgcgtggtggtggccctggatcccgaagaccccgaggtgcagatcagctggttcgtggatggaaagcagatgcagaccgccaagacccaaccccgggaagagcagttcagcggcacctacagggtggtgagtgtgttgcccatcggccaccaggactggctgaaggggaagcaattcacatgcaaggttaataacaaggccctgcccagccccatcgagaggaccatcagcaaggccaggggccaggcccaccagccatctgtgtacgtgctgcccccatctagggaggaactgagcaagaacacagtcagccttacttgcctgatcaaggacttcttcccaccggacatagacgtggagtggcagagtaacggccagcaggagcccgagagcaagtataggaccacaccgccccaactggacgaggacggaagctacttcctctacagcaaattgagcgttgacaaaagcaggtggcagcgaggcgacaccttcatctgcgccgtgatgcacgaggctttgcataaccactacacccaggagagcctgtcccacagccccggatag

SEQ ID NO: 102 - protein, 302 aa, synthetic construct
  REGION 1..302: note = Fusion Protein
FVNQHLCGSHLVEALELVCGERGFHYGGGGGGSGGGGGIVEQCCTSTCSLDQLENYCGGGGGQGGGGQGGGGQGGGGGDCPKCPAPEMLGGPSVFIFPPKPKDTLLIARTPEVTCVVVALDPEDPEVQISWFVDGKQMQTAKTQPREEQFSGTYRVVSVLPIGHQDWLKGKQFTCKVNNKALPSPIERTISKARGQAHQPSVYVLPPSREELSKNTVSLTCLIKDFFPPDIDVEWQSNGQQEPESKYRTTPPQLDEDGSYFLYSKLSVDKSRWQRGDTFICAVMHEALHNHYTQESLSHSPG

SEQ ID NO: 103 - DNA, 966 bp, synthetic construct
  misc_feature 1..966: note = Fusion Protein DNA
  source 1..966: mol_type = other DNA
atggaatggagctgggtctttctcttcttcctgtcagtaacgactggtgtccactccttcgtgaaccagcacctgtgcggctcccacctggtggaagctctggaactcgtgtgcggcgagcggggcttccactacgggggtggcggaggaggttctggtggcggcggaggcatcgtggaacagtgctgcacctccacctgctccctggaccagctggaaaactactgcggtggcggaggtggtcaaggaggcggtggacagggtggaggtgggcagggaggaggcgggggagactgccccaagtgccccgctcccgagatgctgggcggacccagcgtgttcatcttccctcccaagcccaaggacacactgctgatcgccaggaccccggaggtgacctgcgtggtggtggacctggatcccgaagaccccgaggtgcagatcagctggttcgtggatggaaagcagatgcagaccgccaagacccaaccccgggaagagcagttcagcggcacctacagggtggtgagtgtgttgcccatcggccaccaggactggctgaaggggaagcaattcacatgcaaggttaataacaaggccctgcccagccccatcgagaggaccatcagcaaggccaggggccaggcccaccagccatctgtgtacgtgctgcccccatctagggaggaactgagcaagaacacagtcagccttacttgcctgatcaaggacttcttcccaccggacatagacgtggagtggcagagtaacggccagcaggagcccgagagcaagtataggaccacaccgccccaactggacgaggacggaagctacttcctctacagcaaattgagcgttgacaaaagcaggtggcagcgaggcgacaccttcatctgcgccgtgatgcacgaggctttgcataaccactacacccaggagagcctgtcccacagccccggatag

SEQ ID NO: 104 - protein, 302 aa, synthetic construct
  REGION 1..302: note = Fusion Protein
FVNQHLCGSHLVEALELVCGERGFHYGGGGGGSGGGGGIVEQCCTSTCSLDQLENYCGGGGGQGGGGQGGGGQGGGGGDCPKCPAPEMLGGPSVFIFPPKPKDTLLIARTPEVTCVVVDLDPEDPEVQISWFVDGKQMQTAKTQPREEQFSGTYRVVSVLPIGHQDWLKGKQFTCKVNNKALPSPIERTISKARGQAHQPSVYVLPPSREELSKNTVSLTCLIKDFFPPDIDVEWQSNGQQEPESKYRTTPPQLDEDGSYFLYSKLSVDKSRWQRGDTFICAVMHEALHNHYTQESLSHSPG

SEQ ID NO: 105 - DNA, 933 bp, synthetic construct
  misc_feature 1..933: note = Fusion Protein DNA
  source 1..933: mol_type = other DNA
atggaatggagctgggtctttctcttcttcctgtcagtaacgactggtgtccactccttcgtgaaccagcacctgtgcggctccgacctggtggaagctctgtatctcgtgtgcggcgagcggggcttcttctacaccgatcccactggaggcggtccacgcagaggcatcgtggaacagtgctgccactccatctgctccctgtaccagctggaaaactactgcaatggcggaggtggttcaggaggcggtggaggtgagggccccaagtgccccgtgcccgagattcccggtgcccccagcgtgttcatctttcccccaaaacccaaggacaccctgagcatcagcaggacccccgaggtgacctgcctggtggtggacctgggacccgacgacagcaacgtgcagatcacctggttcgtggacaacaccgagatgcacaccgccaagaccaggcctcgggaggagcagttcaacagcacctacagggtggtgagcgtgctgcccatcctgcaccaggactggctgaagggcaaggagttcaagtgcaaggtgaacagcaagagcctgcccagcgccatggagaggaccatcagcaaggccaagggtcagccccacgagccccaagtgtacgtgcttcccccgacccaggaggagttgagcgagaacaaagtgagcgtgacctgcctgatcaagggcttccaccctcccgacatcgccgtggagtgggagatcaccggccagcctgagccggaaaataactaccagaccacccctccacagctggacagcgacggcacctacttcctttacagcaggctgtctgtggaccgaagccattggcaaaggggcaacacctacacctgcagcgtgagccacgaggctctgcacagccaccacacccagaagtctctgacccagagccccggatag

SEQ ID NO: 106 - protein, 291 aa, synthetic construct
  REGION 1..291: note = Fusion Protein
FVNQHLCGSDLVEALYLVCGERGFFYTDPTGGGPRRGIVEQCCHSICSLYQLENYCNGGGGSGGGGGEGPKCPVPEIPGAPSVFIFPPKPKDTLSISRTPEVTCLVVDLGPDDSNVQITWFVDNTEMHTAKTRPREEQFNSTYRVVSVLPILHQDWLKGKEFKCKVNSKSLPSAMERTISKAKGQPHEPQVYVLPPTQEELSENKVSVTCLIKGFHPPDIAVEWEITGQPEPENNYQTTPPQLDSDGTYFLYSRLSVDRSHWQRGNTYTCSVSHEALHSHHTQKSLTQSPG

SEQ ID NO: 107 - DNA, 930 bp, synthetic construct
  misc_feature 1..930: note = Fusion Protein DNA
  source 1..930: mol_type = other DNA
atggaatggagctgggtctttctcttcttcctgtcagtaacgactggtgtccactccttcgtgaaccagcacctgtgcggctccgacctggtggaagctctggctctcgtgtgcggcgagcggggcttcttctacaccgatcccactggaggcggtccacgcagaggcatcgtggaacagtgctgccactccatctgctccctgtaccagctggaaaactactgcaatggtggcggaggatctggcggaggcggtgactgccccaaatgtcctccgcctgagatgctgggtggccctagcatcttcatcttcccgcccaagcccaaggatactctgtccattagcaggacccccgaggtgacctgcctggtggtggacctggggccagacgactctgacgtgcagatcacctggttcgtagacaacacccaggtttacactgccaagaccagtcccagggaggagcagttcaacagcacatacagggtggtgagcgttctgcccatcctgcaccaggactggctgaaaggcaaagagttcaagtgtaaggtgaacagcaagagcctgcccagccccattgaaaggaccatcagcaaggacaagggccagccgcacgagccccaagtctacgtgctgcccccagcacaggaagagctgagcaggaacaaggttagcgtgacatgcctgatcgagggtttctaccccagcgacatcgccgtggagtgggaaatcaccggccaacccgagcccgagaacaactacaggaccactccgccgcaactggacagcgacgggacctacttcttgtatagcaggctgagcgtggaccggagcaggtggcagaggggcaacacctacacttgcagcgtgagccacgaggccttgcacagccaccacactcagaagagtctgacccagagcccgggatag

SEQ ID NO: 108 - protein, 290 aa, synthetic construct
  REGION 1..290: note = Fusion Protein
FVNQHLCGSDLVEALALVCGERGFFYTDPTGGGPRRGIVEQCCHSICSLYQLENYCNGGGGSGGGGDCPKCPPPEMLGGPSIFIFPPKPKDTLSISRTPEVTCLVVDLGPDDSDVQITWFVDNTQVYTAKTSPREEQFNSTYRVVSVLPILHQDWLKGKEFKCKVNSKSLPSPIERTISKDKGQPHEPQVYVLPPAQEELSRNKVSVTCLIEGFYPSDIAVEWEITGQPEPENNYRTTPPQLDSDGTYFLYSRLSVDRSRWQRGNTYTCSVSHEALHSHHTQKSLTQSPG

SEQ ID NO: 109 - DNA, 933 bp, synthetic construct
  misc_feature 1..933: note = Fusion Protein DNA
  source 1..933: mol_type = other DNA
atggaatggagctgggtctttctcttcttcctgtcagtaacgactggtgtccactccttcgtgaaccagcacctgtgcggctccgacctggtggaagctctggctctcgtgtgcggcgagcggggcttcttctacaccgatcccactggaggcggtccacgcagaggcatcgtggaacagtgctgccactccatctgctccctgtaccagctggaaaactactgcaatggcggaggtggtgcaggaggcggtggaggtgagggccccaagtgccccgtgcccgagattcccggtgcccccagcgtgttcatctttcccccaaaacccaaggacaccctgagcatcagcaggacccccgaggtgacctgcctggtggtggacctgggacccgacgacagcaacgtgcagatcacctggttcgtggacaacaccgagatgcacaccgccaagaccaggcctcgggaggagcagttcaacagcacctacagggtggtgagcgtgctgcccatcctgcaccaggactggctgaagggcaaggagttcaagtgcaaggtgaacagcaagagcctgcccagcgccatggagaggaccatcagcaaggccaagggtcagccccacgagccccaagtgtacgtgcttcccccgacccaggaggagttgagcgagaacaaagtgagcgtgacctgcctgatcaagggcttccaccctcccgacatcgccgtggagtgggagatcaccggccagcctgagccggaaaataactaccagaccacccctccacagctggacagcgacggcacctacttcctttacagcaggctgtctgtggaccgaagccattggcaaaggggcaacacctacacctgcagcgtgagccacgaggctctgcacagccaccacacccagaagtctctgacccagagccccggatag

SEQ ID NO: 110 - protein, 291 aa, synthetic construct
  REGION 1..291: note = Fusion Protein
FVNQHLCGSDLVEALALVCGERGFFYTDPTGGGPRRGIVEQCCHSICSLYQLENYCNGGGGAGGGGGEGPKCPVPEIPGAPSVFIFPPKPKDTLSISRTPEVTCLVVDLGPDDSNVQITWFVDNTEMHTAKTRPREEQFNSTYRVVSVLPILHQDWLKGKEFKCKVNSKSLPSAMERTISKAKGQPHEPQVYVLPPTQEELSENKVSVTCLIKGFHPPDIAVEWEITGQPEPENNYQTTPPQLDSDGTYFLYSRLSVDRSHWQRGNTYTCSVSHEALHSHHTQKSLTQSPG

SEQ ID NO: 111 - DNA, 933 bp, synthetic construct
  misc_feature 1..933: note = Fusion Protein DNA
  source 1..933: mol_type = other DNA
atggaatggagctgggtctttctcttcttcctgtcagtaacgactggtgtccactccttcgtgaaccagcacctgtgcggctccgacctggtggaagctctggctctcgtgtgcggcgagcggggcttcttctacaccgatcccactggaggcggtccacgcagaggcatcgtggaacagtgctgccactccatctgctccctgtaccagctggaaaactactgcaatggcggaggtggttcaggaggcggtggaggtgagggccccaagtgccccgtgcccgagattcccggtgcccccagcgtgttcatctttcccccaaaacccaaggacaccctgagcatcagcaggacccccgaggtgacctgcctggtggtggacctgggacccgacgacagcaacgtgcagatcacctggttcgtggacaacaccgagatgcacaccgccaagaccaggcctcgggaggagcagttcaacagcacctacagggtggtgagcgtgctgcccatcctgcaccaggactggctgaagggcaaggagttcaagtgcaaggtgaacagcaagagcctgcccagcgccatggagaggaccatcagcaaggccaagggtcagccccacgagccccaagtgtacgtgcttcccccgacccaggaggagttgagcgagaacaaagtgagcgtgacctgcctgatcaagggcttccaccctcccgacatcgccgtggagtgggagatcaccggccagcctgagccggaaaataactaccagaccacccctccacagctggacagcgacggcacctacttcctttacagcaggctgtctgtggaccgaagccattggcaaaggggcaacacctacacctgcagcgtgagccacgaggctctgcacagccaccacacccagaagtctctgacccagagccccggatag

SEQ ID NO: 112 - protein, 291 aa, synthetic construct
  REGION 1..291: note = Fusion Protein
FVNQHLCGSDLVEALALVCGERGFFYTDPTGGGPRRGIVEQCCHSICSLYQLENYCNGGGGSGGGGGEGPKCPVPEIPGAPSVFIFPPKPKDTLSISRTPEVTCLVVDLGPDDSNVQITWFVDNTEMHTAKTRPREEQFNSTYRVVSVLPILHQDWLKGKEFKCKVNSKSLPSAMERTISKAKGQPHEPQVYVLPPTQEELSENKVSVTCLIKGFHPPDIAVEWEITGQPEPENNYQTTPPQLDSDGTYFLYSRLSVDRSHWQRGNTYTCSVSHEALHSHHTQKSLTQSPG

SEQ ID NO: 113 - DNA, 930 bp, synthetic construct
  misc_feature 1..930: note = Fusion Protein DNA
  source 1..930: mol_type = other DNA
atggaatggagctgggtctttctcttcttcctgtcagtaacgactggtgtccactccttcgtgaaccagcacctgtgcggctcccacctggtggaagctctggctctcgtgtgcggcgagcggggcttcttctacaccgatcccgcaggaggcggtccacgcagaggcatcgtggaacagtgctgcgcatccgtttgctccctgtaccagctggaacactactgcggcggaggtggtgcaggaggcggtggaggtgagggccccaagtgccccgtgcccgagattcccggtgcccccagcgtgttcatctttcccccaaaacccaaggacaccctgagcatcagcaggacccccgaggtgacctgcctggtggtggacctgggacccgacgacagcaacgtgcagatcacctggttcgtggacaacaccgagatgcacaccgccaagaccaggcctcgggaggagcagttcaacagcacctacagggtggtgagcgtgctgcccatcctgcaccaggactggctgaagggcaaggagttcaagtgcaaggtgaacagcaagagcctgcccagcgccatggagaggaccatcagcaaggccaagggtcagccccacgagccccaagtgtacgtgcttcccccgacccaggaggagttgagcgagaacaaagtgagcgtgacctgcctgatcaagggcttccaccctcccgacatcgccgtggagtgggagatcaccggccagcctgagccggaaaataactaccagaccacccctccacagctggacagcgacggcacctacttcctttacagcaggctgtctgtggaccgaagccattggcaaaggggcaacacctacacctgcagcgtgagccacgaggctctgcacagccaccacacccagaagtctctgacccagagccccggatag

SEQ ID NO: 114 - protein, 289 aa, synthetic construct
  REGION 1..289: note = Fusion Protein
FVNQHLCGSHLVEALALVCGERGFFYTDPAGGGPRRGIVEQCCASVCSLYQLEHYCGGGGAGGGGGEGPKCPVPEIPGAPSVFIFPPKPKDTLSISRTPEVTCLVVDLGPDDSNVQITWFVDNTEMHTAKTRPREEQFNSTYRVVSVLPILHQDWLKGKEFKCKVNSKSLPSAMERTISKAKGQPHEPQVYVLPPTQEELSENKVSVTCLIKGFHPPDIAVEWEITGQPEPENNYQTTPPQLDSDGTYFLYSRLSVDRSHWQRGNTYTCSVSHEALHSHHTQKSLTQSP

SEQ ID NO: 115 - DNA, 930 bp, synthetic construct
  misc_feature 1..930: note = Fusion Protein DNA
  source 1..930: mol_type = other DNA
atggaatggagctgggtctttctcttcttcctgtcagtaacgactggtgtccactccttcgtgaaccagcacctgtgcggctcccacctggtggaagctctggctctcgtgtgcggcgagcggggcttcttctacaccgatcccgcaggaggcggtccacgcagaggcatcgtggaacagtgctgcgcatccgtttgctccctgtaccagctggaacactactgcggcggaggtggtgcaggaggcggtggaggtgagggccccaagtgccccgtgcccgagattcccggtgcccccagcgtgttcatctttcccccaaaacccaaggacaccctgagcatcagcaggacccccgaggtgacctgcctggtggtggacctgggacccgacgacagcaacgtgcagatcacctggttcgtggacaacaccgagatgcacaccgccaagaccaggcctcgggaggagcagttcagcagcacctacagggtggtgagcgtgctgcccatcctgcaccaggactggctgaagggcaaggagttcaagtgcaaggtgaacagcaagagcctgcccagcgccatggagaggaccatcagcaaggccaagggtcagccccacgagccccaagtgtacgtgcttcccccgacccaggaggagttgagcgagaacaaagtgagcgtgacctgcctgatcaagggcttccaccctcccgacatcgccgtggagtgggagatcaccggccagcctgagccggaaaataactaccagaccacccctccacagctggacagcgacggcacctacttcctttacagcaggctgtctgtggaccgaagccattggcaaaggggcaacacctacacctgcagcgtgagccacgaggctctgcacagccaccacacccagaagtctctgacccagagccccggatag

SEQ ID NO: 116 - protein, 290 aa, synthetic construct
  REGION 1..290: note = Fusion Protein
FVNQHLCGSHLVEALALVCGERGFFYTDPAGGGPRRGIVEQCCASVCSLYQLEHYCGGGGAGGGGGEGPKCPVPEIPGAPSVFIFPPKPKDTLSISRTPEVTCLVVDLGPDDSNVQITWFVDNTEMHTAKTRPREEQFSSTYRVVSVLPILHQDWLKGKEFKCKVNSKSLPSAMERTISKAKGQPHEPQVYVLPPTQEELSENKVSVTCLIKGFHPPDIAVEWEITGQPEPENNYQTTPPQLDSDGTYFLYSRLSVDRSHWQRGNTYTCSVSHEALHSHHTQKSLTQSPG

SEQ ID NO: 117 - DNA, 927 bp, synthetic construct
  misc_feature 1..927: note = Fusion Protein DNA
  source 1..927: mol_type = other DNA
atggaatggagctgggtctttctcttcttcctgtcagtaacgactggtgtccactccttcgtgaaccagcacctgtgcggaagccacctggtggaggccttggccctggtgtgcggcgagaggggcttcttctacaccgaccccgctggtggcggacctaggaggggcatcgtggagcagtgctgcgccagcgtgtgcagcctgtaccagttggaacactactgcggaggtggcggagccggaggcgggggagactgccccaaatgtcctccgcctgagatgctgggtggccctagcatcttcatcttcccgcccaagcccaaggatactctgtccattagcaggacccccgaggtgacctgcctggtggtggcactggggccagacgactctgacgtgcagatcacctggttcgtagacaacacccaggtttacactgccaagaccagtcccagggaggagcagttcagcagcacatacagggtggtgagcgttctgcccatcctgcaccaggactggctgaaaggcaaagagttcaagtgtaaggtgaacagcaagagcctgcccagccccattgaaaggaccatcagcaaggacaagggccagccgcacgagccccaagtctacgtgctgcccccagcacaggaagagctgagcaggaacaaggttagcgtgacatgcctgatcgagggtttctaccccagcgacatcgccgtggagtgggaaatcaccggccaacccgagcccgagaacaactacaggaccactccgccgcaactggacagcgacgggacctacttcttgtatagcaggctgagcgtggaccggagcaggtggcagaggggcaacacctacacttgcagcgtgagccacgaggccttgcacagccaccacactcagaagagtctgacccagagcccgggatag

SEQ ID NO: 118 - protein, 289 aa, synthetic construct
  REGION 1..289: note = Fusion Protein
FVNQHLCGSHLVEALALVCGERGFFYTDPAGGGPRRGIVEQCCASVCSLYQLEHYCGGGGAGGGGDCPKCPPPEMLGGPSIFIFPPKPKDTLSISRTPEVTCLVVALGPDDSDVQITWFVDNTQVYTAKTSPREEQFSSTYRVVSVLPILHQDWLKGKEFKCKVNSKSLPSPIERTISKDKGQPHEPQVYVLPPAQEELSRNKVSVTCLIEGFYPSDIAVEWEITGQPEPENNYRTTPPQLDSDGTYFLYSRLSVDRSRWQRGNTYTCSVSHEALHSHHTQKSLTQSPG

SEQ ID NO: 119 - DNA, 168 bp, synthetic construct
  misc_feature 1..168: note = Ins Polypeptide DNA
  source 1..168: mol_type = other DNA
ttcgtgaaccagcacctgtgcggaagccacctggtggaggccttggccctggtgtgcggcgagaggggcttcttctacaccgaccccgctggtggcggacctaggaggggcatcgtggagcagtgctgcgccagcgtgtgcagcctgtaccagttggaacactactgc

SEQ ID NO: 120 - protein, 56 aa, synthetic construct
  REGION 1..56: note = Ins Polypeptide
FVNQHLCGSHLVEALALVCGERGFFYTDPAGGGPRRGIVEQCCASVCSLYQLEHYC

SEQ ID NO: 121 - DNA, 969 bp, synthetic construct
  misc_feature 1..969: note = Fusion Protein DNA
  source 1..969: mol_type = other DNA
atggaatggagctgggtctttctcttcttcctgtcagtaacgactggtgtccactccttcgtgaaccagcacctgtgcggctcccacctggtggaagctctggaactcgtgtgcggcgagcggggcttccactacgggggtggcggaggaggttctggtggcggcggaggcatcgtggaacagtgctgcacctccacctgctccctggaccagctggaaaactactgcggtggcggaggtggtcaaggaggcggtggacagggtggaggtgggcagggaggaggcgggggaggtgagggccccaagtgccccgtgcccgagattcccggtgcccccagcgtgttcatctttcccccaaaacccaaggacaccctgagcatcagcaggacccccgaggtgacctgcctggtggtggacctgggacccgacgacagcaacgtgcagatcacctggttcgtggacaacaccgagatgcacaccgccaagaccaggcctcgggaggagcagttcaacagcacctacagggtggtgagcgtgctgcccatcctgcaccaggactggctgaagggcaaggagttcaagtgcaaggtgaacagcaagagcctgcccagcgccatggagaggaccatcagcaaggccaagggtcagccccacgagccccaagtgtacgtgcttcccccgacccaggaggagttgagcgagaacaaagtgagcgtgacctgcctgatcaagggcttccaccctcccgacatcgccgtggagtgggagatcaccggccagcctgagccggaaaataactaccagaccacccctccacagctggacagcgacggcacctacttcctttacagcaggctgtctgtggaccgaagccattggcaaaggggcaacacctacacctgcagcgtgagccacgaggctctgcacagccaccacacccagaagtctctgacccagagccccggatag

SEQ ID NO: 122 - protein, 303 aa, synthetic construct
  REGION 1..303: note = Fusion Protein
FVNQHLCGSHLVEALELVCGERGFHYGGGGGGSGGGGGIVEQCCTSTCSLDQLENYCGGGGGQGGGGQGGGGQGGGGGGEGPKCPVPEIPGAPSVFIFPPKPKDTLSISRTPEVTCLVVDLGPDDSNVQITWFVDNTEMHTAKTRPREEQFNSTYRVVSVLPILHQDWLKGKEFKCKVNSKSLPSAMERTISKAKGQPHEPQVYVLPPTQEELSENKVSVTCLIKGFHPPDIAVEWEITGQPEPENNYQTTPPQLDSDGTYFLYSRLSVDRSHWQRGNTYTCSVSHEALHSHHTQKSLTQSPG

SEQ ID NO: 123 - DNA, 966 bp, synthetic construct
  misc_feature 1..966: note = Fusion Protein DNA
  source 1..966: mol_type = other DNA
atggaatggagctgggtctttctcttcttcctgtcagtaacgactggtgtccactccttcgtgaaccagcacctgtgcggctcccacctggtggaagctctggaactcgtgtgcggcgagcggggcttccactacgggggtggcggaggaggttctggtggcggcggaggcatcgtggaacagtgctgcacctccacctgctccctggaccagctggaaaactactgcggtggcggaggtggtcaaggaggcggtggacagggtggaggtgggcagggaggaggcgggggagactgccccaaatgtcctccgcctgagatgctgggtggccctagcatcttcatcttcccgcccaagcccaaggatactctgtccattagcaggacccccgaggtgacctgcctggtggtggacctggggccagacgactctgacgtgcagatcacctggttcgtagacaacacccaggtttacactgccaagaccagtcccagggaggagcagttcagcagcacatacagggtggtgagcgttctgcccatcctgcaccaggactggctgaaaggcaaagagttcaagtgtaaggtgaacagcaagagcctgcccagccccattgaaaggaccatcagcaaggacaagggccagccgcacgagccccaagtctacgtgctgcccccagcacaggaagagctgagcaggaacaaggttagcgtgacatgcctgatcgagggtttctaccccagcgacatcgccgtggagtgggaaatcaccggccaacccgagcccgagaacaactacaggaccactccgccgcaactggacagcgacgggacctacttcttgtatagcaggctgagcgtggaccggagcaggtggcagaggggcaacacctacacttgcagcgtgagccacgaggccttgcacagccaccacactcagaagagtctgacccagagcccgggatag

SEQ ID NO: 124 - protein, 302 aa, synthetic construct
  REGION 1..302: note = Fusion Protein
FVNQHLCGSHLVEALELVCGERGFHYGGGGGGSGGGGGIVEQCCTSTCSLDQLENYCGGGGGQGGGGQGGGGQGGGGGDCPKCPPPEMLGGPSIFIFPPKPKDTLSISRTPEVTCLVVDLGPDDSDVQITWFVDNTQVYTAKTSPREEQFSSTYRVVSVLPILHQDWLKGKEFKCKVNSKSLPSPIERTISKDKGQPHEPQVYVLPPAQEELSRNKVSVTCLIEGFYPSDIAVEWEITGQPEPENNYRTTPPQLDSDGTYFLYSRLSVDRSRWQRGNTYTCSVSHEALHSHHTQKSLTQSPG

SEQ ID NO: 125 - protein, 57 aa, synthetic construct
  REGION 1..57: note = Ins Polypeptide
FVNQHLCGSHLVEALALVCGERGFFYTDPTGGGPRRGIVEQCCTSICSLYQLENYCN

SEQ ID NO: 126 - protein, 10 aa, synthetic construct
  REGION 1..10: note = Linker
GGGGGAGGGG

SEQ ID NO: 127 - protein, 19 aa, synthetic construct
  REGION 1..19: note = Linker
GGGGSGGGGSGGGGSGGGG

SEQ ID NO: 128 - protein, 19 aa, synthetic construct
  REGION 1..19: note = Linker
GGGGKGGGGKGGGGKGGGG

SEQ ID NO: 129 - protein, 21 aa, synthetic construct
  REGION 1..21: note = Linker
GGGGGAGGGGAGGGGAGGGGG

SEQ ID NO: 130 - protein, 21 aa, synthetic construct
  REGION 1..21: note = Linker
SGGGGQGGGGQGGGGQGGGGG

SEQ ID NO: 131 - protein, 21 aa, synthetic construct
  REGION 1..21: note = Linker
HGGGGQGGGGQGGGGQGGGGG

SEQ ID NO: 132 - protein, 22 aa, synthetic construct
  REGION 1..22: note = Linker
PGGGGGQGGGGQGGGGQGGGGG

SEQ ID NO: 133 - protein, 11 aa, synthetic construct
  REGION 1..11: note = C-Chain
GGGGGGSGGGG